European Patent Application EP 4 707 293 A1, published March 11, 2026. Title: RSV F蛋白的突变体. Applicant: 国药中生生物技术研究院有限公司. The sequence listing filed with the application follows.

SEQUENCE LISTING (166 sequences)

SEQ ID NO: 1 - protein, 574 aa, Respiratory syncytial virus
MELLILKANAITTILTAVTFCFASGQNITEEFYQSTCSAVSKGYLSALRTGWYTSVITIELSNIKENKCNGTDAKVKLIKQELDKYKNAVTELQLLMQSTPATNNRARRELPRFMNYTLNNAKKTNVTLSKKRKRRFLGFLLGVGSAIASGVAVSKVLHLEGEVNKIKSALLSTNKAVVSLSNGVSVLTSKVLDLKNYIDKQLLPIVNKQSCSISNIETVIEFQQKNNRLLEITREFSVNAGVTTPVSTYMLTNSELLSLINDMPITNDQKKLMSNNVQIVRQQSYSIMSIIKEEVLAYVVQLPLYGVIDTPCWKLHTSPLCTTNTKEGSNICLTRTDRGWYCDNAGSVSFFPQAETCKVQSNRVFCDTMNSLTLPSEVNLCNVDIFNPKYDCKIMTSKTDVSSSVITSLGAIVSCYGKTKCTASNKNRGIIKTFSNGCDYVSNKGVDTVSVGNTLYYVNKQEGKSLYVKGEPIINFYDPLVFPSDEFDASISQVNEKINQSLAFIRKSDELLHNVNAGKSTTNIMITTIIIVIIVILLSLIAVGLLLYCKARSTPVTLSKDQLSGINNIAFSN

SEQ ID NO: 2 - protein, 574 aa, Respiratory syncytial virus
MELLILKANAITTILTAVTFCFASGQNITEEFYQSTCSAVSKGYLSALRTGWYTSVITIELSNIKENKCNGTDAKVKLIKQELDKYKNAVTELQLLMQSTPPTNNRARRELPRFMNYTLNNAKKTNVTLSKKRKRRFLGFLLGVGSAIASGVAVSKVLHLEGEVNKIKSALLSTNKAVVSLSNGVSVLTSKVLDLKNYIDKQLLPIVNKQSCSISNIETVIEFQQKNNRLLEITREFSVNAGVTTPVSTYMLTNSELLSLINDMPITNDQKKLMSNNVQIVRQQSYSIMSIIKEEVLAYVVQLPLYGVIDTPCWKLHTSPLCTTNTKEGSNICLTRTDRGWYCDNAGSVSFFPQAETCKVQSNRVFCDTMNSLTLPSEINLCNVDIFNPKYDCKIMTSKTDVSSSVITSLGAIVSCYGKTKCTASNKNRGIIKTFSNGCDYVSNKGMDTVSVGNTLYYVNKQEGKSLYVKGEPIINFYDPLVFPSDEFDASISQVNEKINQSLAFIRKSDELLHNVNAGKSTTNIMITTIIIVIIVILLSLIAVGLLLYCKARSTPVTLSKDQLSGINNIAFSN

SEQ ID NO: 3 - protein, 574 aa, Respiratory syncytial virus
MELPIIKTNAITAILAAVTLCFASSQNITEEFYQSTCSAVSKGYLSALRTGWYTSVITIELSNIKENKCNGTDAKVKLIKQELDKYKNAVTELQLLMQSTPAANSRARRELPRFMNYTLNNTKNTNVTLSKKRKRRFLGFLLGVGSAIASGIAVSKVLHLEGEVNKIKSALLSTNKAVVSLSNGVSVLTSKVLDLKNYIDKQLLPIVNKQSCSISNIETVIEFQQKNNRLLEITREFSVNAGVTTPVSTYMLTNSELLSLINDMPITNDQKKLMSSNVQIVRQQSYSIMSIIKEEVLAYVVQLPLYGVIDTPCWKLHTSPLCTTNTKEGSNICLTRTDRGWYCDNAGSVSFFPQAETCKVQSNRVFCDTMNSLTLPSEVNLCNIDIFNPKYDCKIMTSKTDVSSSVITSLGAIVSCYGKTKCTASNKNRGIIKTFSNGCDYVSNKGVDTVSVGNTLYYVNKQEGKSLYVKGEPIINFYDPLVFPSDEFDASISQVNEKINQSLAFIRKSDELLHNVNAGKSTTNIMITTIIIVIIVILLALIAVGLLLYCKARSTPVTLSKDQLSGINNIAFSN

SEQ ID NO: 4 - protein, 574 aa, Respiratory syncytial virus
MELLIHRSSAIFLTLAINALHLTSSQNITEEFYQSTCSAVSRGYLSALRTGWYTSVITIELSNIKETKCNGTDTKVKLIKQELDKYKNAVTELQLLMQNTPAVNNRARREAPQYMNYTINTTKNLNVSISKKRKRRFLGFLLGVGSAIASGIAVSKVLHLEGEVNKIKNALQLTNKAVVSLSNGVSVLTSRVLDLKNYINNQLLPMVNRQSCRISNIETVIEFQQKNSRLLEITREFSVNAGVTTPLSTYMLTNSELLSLINDMPITNDQKKLMSSNVQIVRQQSYSIMSIIKEEVLAYVVQLPIYGVIDTPCWKLHTSPLCTTNIKEGSNICLTRTDRGWYCDNAGSVSFFPQADTCKVQSNRVFCDTMNSLTLPSEVSLCNTDIFNSKYDCKIMTSKTDISSSVITSLGAIVSCYGKTKCTASNKNRGIIKTFSNGCDYVSNKGVDTVSVGNTLYYVNKLEGKNLYVKGEPIINYYDPLVFPSDEFDASISQVNEKINQSLAFIRRSDELLHNVNTGKSTTNIMITAIIIVIIVVLLSLIAIGLLLYCKAKNTPVTLSKDQLSGINNIAFSK

SEQ ID NO: 5 - protein, 574 aa, Respiratory syncytial virus
MELLIHRSSAIFLTLAINALYLTSSQNITEEFYQSTCSAVSRGYFSALRTGWYTSVITIELSNIKETKCNGTDTKVKLIKQELDKYKNAVTELQLLMQNTPAANNRARREAPQYMNYTINTTKNLNVSISKKRKRRFLGFLLGVGSAIASGIAVSKVLHLEGEVNKIKNALLSTNKAVVSLSNGVSVLTSKVLDLKNYINNQLLPIVNQQSCRISNIETVIEFQQKNSRLLEITREFSVNAGVTTPLSTYMLTNSELLSLINDMPITNDQKKLMSSNVQIVRQQSYSIMSIIKEEVLAYVVQLPIYGVIDTPCWKLHTSPLCTTNIKEGSNICLTRTDRGWYCDNAGSVSFFPQADTCKVQSNRVFCDTMNSLTLPSEVSLCNTDIFNSKYDCKIMTSKTDISSSVITSLGAIVSCYGKTKCTASNKNRGIIKTFSNGCDYVSNKGVDTVSVGNTLYYVNKLEGKNLYVKGEPIINYYDPLVFPSDEFDASISQVNEKINQSLAFIRRSDELLHNVNTGKSTTNIMITAIIIVIIVVLLSLIAIGLLLYCKAKNTPVTLSKDQLSGINNIAFSK

SEQ ID NO: 6 - protein, 574 aa, Respiratory syncytial virus
MELLIHRSSAIFLTLAVNALYLTSSQNITEEFYQSTCSAVSRGYFSALRTGWYTSVITIELSNIKETKCNGTDTKVKLIKQELDKYKNAVTELQLLMQNTPAANNRARREAPQYMNYTINTTKNLNVSISKKRKRRFLGFLLGVGSAIASGIAVSKVLHLEGEVNKIKNALLSTNKAVVSLSNGVSVLTSKVLDLKNYINNRLLPIVNQQSCRISNIETVIEFQQMNSRLLEITREFSVNAGVTTPLSTYMLTNSELLSLINDMPITNDQKKLMSSNVQIVRQQSYSIMSIIKEEVLAYVVQLPIYGVIDTPCWKLHTSPLCTTNIKEGSNICLTRTDRGWYCDNAGSVSFFPQADTCKVQSNRVFCDTMNSLTLPSEVSLCNTDIFNSKYDCKIMTSKTDISSSVITSLGAIVSCYGKTKCTASNKNRGIIKTFSNGCDYVSNKGVDTVSVGNTLYYVNKLEGKNLYVKGEPIINYYDPLVFPSDEFDASISQVNEKINQSLAFIRRSDELLHNVNTGKSTTNIMITTIIIVIIVVLLSLIAIGLLLYCKAKNTPVTLSKDQLSGINNIAFSK

SEQ ID NO: 7 - protein, 488 aa, synthetic construct
QNITEEFYQSTCSAVSKGYLSALRTGWYTSVITIELSNIKENKCNGTDAKVKLIKQELDKYKNAVTELQLLMQSTPATNNRARRELPRFMNYTLNNAKKTNVTLSKKRKRRFLGFLLGVGSAIASGVAVSKVLHLEGEVNKIKSALLSTNKAVVSLSNGVSVLTSKVLDLKNYIDKQLLPIVNKQSCSISNIETVIEFQQKNNRLLEITREFSVNAGVTTPVSTYMLTNSELLSLINDMPITNDQKKLMSNNVQIVRQQSYSIMSIIKEEVLAYVVQLPLYGVIDTPCWKLHTSPLCTTNTKEGSNICLTRTDRGWYCDNAGSVSFFPQAETCKVQSNRVFCDTMNSLTLPSEVNLCNVDIFNPKYDCKIMTSKTDVSSSVITSLGAIVSCYGKTKCTASNKNRGIIKTFSNGCDYVSNKGVDTVSVGNTLYYVNKQEGKSLYVKGEPIINFYDPLVFPSDEFDASISQVNEKINQSLAFIRKSDELL

SEQ ID NO: 8 - protein, 504 aa, synthetic construct
QNITEEFYQSTCSAVSKGYLSALRTGWYTSVITIELSNIKENKCNGTDAKVKLIKQELDKYKNAVTELQLLMQSTPATNNRARRELPRFMNYTLNNAKKTNVTLSKKRKRRFLGFLLGVGSAIASGVAVSKVLHLEGEVNKIKSALLSTNKAVVSLSNGVSVLTSKVLDLKNYIDKQLLPIVNKQSCSISNIETVIEFQQKNNRLLEITREFSVNAGVTTPVSTYMLTNSELLSLINDMPITNDQKKLMSNNVQIVRQQSYSIMSIIKEEVLAYVVQLPLYGVIDTPCWKLHTSPLCTTNTKEGSNICLTRTDRGWYCDNAGSVSFFPQAETCKVQSNRVFCDTMNSLTLPSEVNLCNVDIFNPKYDCKIMTSKTDVSSSVITSLGAIVSCYGKTKCTASNKNRGIIKTFSNGCDYVSNKGVDTVSVGNTLYYVNKQEGKSLYVKGEPIINFYDPLVFPSDEFDASISQVNEKINQSLAFIRKSDELLHNVNAGKSTTNIMITT

SEQ ID NO: 9 - protein, 488 aa, synthetic construct
QNITEEFYQSTCSAVSKGYLSALRTGWYTSVITIELSNIKENKCNGTDAKVKLIKQELDKYKNAVTELQLLMQSTPATNNQARRELPRFMNYTLNNAKKTNVTLSKKRKSSFLGFLLGVGSAIASGVAVSKVLHLEGEVNKIKSALLSTNKAVVSLSNGVSVLTSKVLDLKNYIDKQLLPIVNKQSCSISNIETVIEFQQKNNRLLEITREFSVNAGVTTPVSTYMLTNSELLSLINDMPITNDQKKLMSNNVQIVRQQSYSIMSIIKEEVLAYVVQLPLYGVIDTPCWKLHTSPLCTTNTKEGSNICLTRTDRGWYCDNAGSVSFFPQAETCKVQSNRVFCDTMNSLTLPSEVNLCNVDIFNPKYDCKIMTSKTDVSSSVITSLGAIVSCYGKTKCTASNKNRGIIKTFSNGCDYVSNKGVDTVSVGNTLYYVNKQEGKSLYVKGEPIINFYDPLVFPSDEFDASISQVNEKINQSLAFIRKSDELL

SEQ ID NO: 10 - protein, 84 aa, synthetic construct
QNITEEFYQSTCSAVSKGYLSALRTGWYTSVITIELSNIKENKCNGTDAKVKLIKQELDKYKNAVTELQLLMQSTPATNNRARR

SEQ ID NO: 11 - protein, 377 aa, synthetic construct
FLGFLLGVGSAIASGVAVSKVLHLEGEVNKIKSALLSTNKAVVSLSNGVSVLTSKVLDLKNYIDKQLLPIVNKQSCSISNIETVIEFQQKNNRLLEITREFSVNAGVTTPVSTYMLTNSELLSLINDMPITNDQKKLMSNNVQIVRQQSYSIMSIIKEEVLAYVVQLPLYGVIDTPCWKLHTSPLCTTNTKEGSNICLTRTDRGWYCDNAGSVSFFPQAETCKVQSNRVFCDTMNSLTLPSEVNLCNVDIFNPKYDCKIMTSKTDVSSSVITSLGAIVSCYGKTKCTASNKNRGIIKTFSNGCDYVSNKGVDTVSVGNTLYYVNKQEGKSLYVKGEPIINFYDPLVFPSDEFDASISQVNEKINQSLAFIRKSDELL

SEQ ID NO: 12 - protein, 466 aa, synthetic construct
QNITEEFYQSTCSAVSKGYLSALRTGWYTSVITIELSNIKENKCNGTDAKVKLIKQELDKYKNAVTELQLLMQSTPATNNQARGSGSGRSLGFLLGVGSAIASGVAVSKVLHLEGEVNKIKSALLSTNKAVVSLSNGVSVLTSKVLDLKNYIDKQLLPIVNKQSCSISNIETVIEFQQKNNRLLEITREFSVNAGVTTPVSTYMLTNSELLSLINDMPITNDQKKLMSNNVQIVRQQSYSIMSIIKEEVLAYVVQLPLYGVIDTPCWKLHTSPLCTTNTKEGSNICLTRTDRGWYCDNAGSVSFFPQAETCKVQSNRVFCDTMNSLTLPSEVNLCNVDIFNPKYDCKIMTSKTDVSSSVITSLGAIVSCYGKTKCTASNKNRGIIKTFSNGCDYVSNKGVDTVSVGNTLYYVNKQEGKSLYVKGEPIINFYDPLVFPSDEFDASISQVNEKINQSLAFIRKSDELL

SEQ ID NO: 13 - protein, 449 aa, synthetic construct
QNITEEFYQSTCSAVSKGYLSALRTGWYTSVITIELSNIKENKCNGTDAKVKLIKQELDKYKNAVTELQLLMQSTPATGSGSAIASGVAVSKVLHLEGEVNKIKSALLSTNKAVVSLSNGVSVLTSKVLDLKNYIDKQLLPIVNKQSCSISNIETVIEFQQKNNRLLEITREFSVNAGVTTPVSTYMLTNSELLSLINDMPITNDQKKLMSNNVQIVRQQSYSIMSIIKEEVLAYVVQLPLYGVIDTPCWKLHTSPLCTTNTKEGSNICLTRTDRGWYCDNAGSVSFFPQAETCKVQSNRVFCDTMNSLTLPSEVNLCNVDIFNPKYDCKIMTSKTDVSSSVITSLGAIVSCYGKTKCTASNKNRGIIKTFSNGCDYVSNKGVDTVSVGNTLYYVNKQEGKSLYVKGEPIINFYDPLVFPSDEFDASISQVNEKINQSLAFIRKSDELL

SEQ ID NO: 14 - protein, 488 aa, synthetic construct
QNITEEFYQSTCSAVSKGYLSALRTGWYTSVITIELSNIKENKCNGTDAKVKLIKQELDKYKNAVTELQLLMQSTPPTNNRARRELPRFMNYTLNNAKKTNVTLSKKRKRRFLGFLLGVGSAIASGVAVSKVLHLEGEVNKIKSALLSTNKAVVSLSNGVSVLTSKVLDLKNYIDKQLLPIVNKQSCSISNIETVIEFQQKNNRLLEITREFSVNAGVTTPVSTYMLTNSELLSLINDMPITNDQKKLMSNNVQIVRQQSYSIMSIIKEEVLAYVVQLPLYGVIDTPCWKLHTSPLCTTNTKEGSNICLTRTDRGWYCDNAGSVSFFPQAETCKVQSNRVFCDTMNSLTLPSEINLCNVDIFNPKYDCKIMTSKTDVSSSVITSLGAIVSCYGKTKCTASNKNRGIIKTFSNGCDYVSNKGMDTVSVGNTLYYVNKQEGKSLYVKGEPIINFYDPLVFPSDEFDASISQVNEKINQSLAFIRKSDELL

SEQ ID NO: 15 - protein, 504 aa, synthetic construct
QNITEEFYQSTCSAVSKGYLSALRTGWYTSVITIELSNIKENKCNGTDAKVKLIKQELDKYKNAVTELQLLMQSTPPTNNRARRELPRFMNYTLNNAKKTNVTLSKKRKRRFLGFLLGVGSAIASGVAVSKVLHLEGEVNKIKSALLSTNKAVVSLSNGVSVLTSKVLDLKNYIDKQLLPIVNKQSCSISNIETVIEFQQKNNRLLEITREFSVNAGVTTPVSTYMLTNSELLSLINDMPITNDQKKLMSNNVQIVRQQSYSIMSIIKEEVLAYVVQLPLYGVIDTPCWKLHTSPLCTTNTKEGSNICLTRTDRGWYCDNAGSVSFFPQAETCKVQSNRVFCDTMNSLTLPSEINLCNVDIFNPKYDCKIMTSKTDVSSSVITSLGAIVSCYGKTKCTASNKNRGIIKTFSNGCDYVSNKGMDTVSVGNTLYYVNKQEGKSLYVKGEPIINFYDPLVFPSDEFDASISQVNEKINQSLAFIRKSDELLHNVNAGKSTTNIMITT

SEQ ID NO: 16 - protein, 488 aa, synthetic construct
QNITEEFYQSTCSAVSKGYLSALRTGWYTSVITIELSNIKENKCNGTDAKVKLIKQELDKYKNAVTELQLLMQSTPPTNNQARRELPRFMNYTLNNAKKTNVTLSKKRKSSFLGFLLGVGSAIASGVAVSKVLHLEGEVNKIKSALLSTNKAVVSLSNGVSVLTSKVLDLKNYIDKQLLPIVNKQSCSISNIETVIEFQQKNNRLLEITREFSVNAGVTTPVSTYMLTNSELLSLINDMPITNDQKKLMSNNVQIVRQQSYSIMSIIKEEVLAYVVQLPLYGVIDTPCWKLHTSPLCTTNTKEGSNICLTRTDRGWYCDNAGSVSFFPQAETCKVQSNRVFCDTMNSLTLPSEINLCNVDIFNPKYDCKIMTSKTDVSSSVITSLGAIVSCYGKTKCTASNKNRGIIKTFSNGCDYVSNKGMDTVSVGNTLYYVNKQEGKSLYVKGEPIINFYDPLVFPSDEFDASISQVNEKINQSLAFIRKSDELL

SEQ ID NO: 17 - protein, 84 aa, synthetic construct
QNITEEFYQSTCSAVSKGYLSALRTGWYTSVITIELSNIKENKCNGTDAKVKLIKQELDKYKNAVTELQLLMQSTPPTNNRARR

SEQ ID NO: 18 - protein, 377 aa, synthetic construct
FLGFLLGVGSAIASGVAVSKVLHLEGEVNKIKSALLSTNKAVVSLSNGVSVLTSKVLDLKNYIDKQLLPIVNKQSCSISNIETVIEFQQKNNRLLEITREFSVNAGVTTPVSTYMLTNSELLSLINDMPITNDQKKLMSNNVQIVRQQSYSIMSIIKEEVLAYVVQLPLYGVIDTPCWKLHTSPLCTTNTKEGSNICLTRTDRGWYCDNAGSVSFFPQAETCKVQSNRVFCDTMNSLTLPSEINLCNVDIFNPKYDCKIMTSKTDVSSSVITSLGAIVSCYGKTKCTASNKNRGIIKTFSNGCDYVSNKGMDTVSVGNTLYYVNKQEGKSLYVKGEPIINFYDPLVFPSDEFDASISQVNEKINQSLAFIRKSDELL

SEQ ID NO: 19 - protein, 466 aa, synthetic construct
QNITEEFYQSTCSAVSKGYLSALRTGWYTSVITIELSNIKENKCNGTDAKVKLIKQELDKYKNAVTELQLLMQSTPPTNNQARGSGSGRSLGFLLGVGSAIASGVAVSKVLHLEGEVNKIKSALLSTNKAVVSLSNGVSVLTSKVLDLKNYIDKQLLPIVNKQSCSISNIETVIEFQQKNNRLLEITREFSVNAGVTTPVSTYMLTNSELLSLINDMPITNDQKKLMSNNVQIVRQQSYSIMSIIKEEVLAYVVQLPLYGVIDTPCWKLHTSPLCTTNTKEGSNICLTRTDRGWYCDNAGSVSFFPQAETCKVQSNRVFCDTMNSLTLPSEINLCNVDIFNPKYDCKIMTSKTDVSSSVITSLGAIVSCYGKTKCTASNKNRGIIKTFSNGCDYVSNKGMDTVSVGNTLYYVNKQEGKSLYVKGEPIINFYDPLVFPSDEFDASISQVNEKINQSLAFIRKSDELL

SEQ ID NO: 20 - protein, 449 aa, synthetic construct
QNITEEFYQSTCSAVSKGYLSALRTGWYTSVITIELSNIKENKCNGTDAKVKLIKQELDKYKNAVTELQLLMQSTPPTGSGSAIASGVAVSKVLHLEGEVNKIKSALLSTNKAVVSLSNGVSVLTSKVLDLKNYIDKQLLPIVNKQSCSISNIETVIEFQQKNNRLLEITREFSVNAGVTTPVSTYMLTNSELLSLINDMPITNDQKKLMSNNVQIVRQQSYSIMSIIKEEVLAYVVQLPLYGVIDTPCWKLHTSPLCTTNTKEGSNICLTRTDRGWYCDNAGSVSFFPQAETCKVQSNRVFCDTMNSLTLPSEINLCNVDIFNPKYDCKIMTSKTDVSSSVITSLGAIVSCYGKTKCTASNKNRGIIKTFSNGCDYVSNKGMDTVSVGNTLYYVNKQEGKSLYVKGEPIINFYDPLVFPSDEFDASISQVNEKINQSLAFIRKSDELL

SEQ ID NO: 21 - protein, 488 aa, synthetic construct
QNITEEFYQSTCSAVSKGYLSALRTGWYTSVITIELSNIKENKCNGTDAKVKLIKQELDKYKNAVTELQLLMQSTPAANSRARRELPRFMNYTLNNTKNTNVTLSKKRKRRFLGFLLGVGSAIASGIAVSKVLHLEGEVNKIKSALLSTNKAVVSLSNGVSVLTSKVLDLKNYIDKQLLPIVNKQSCSISNIETVIEFQQKNNRLLEITREFSVNAGVTTPVSTYMLTNSELLSLINDMPITNDQKKLMSSNVQIVRQQSYSIMSIIKEEVLAYVVQLPLYGVIDTPCWKLHTSPLCTTNTKEGSNICLTRTDRGWYCDNAGSVSFFPQAETCKVQSNRVFCDTMNSLTLPSEVNLCNIDIFNPKYDCKIMTSKTDVSSSVITSLGAIVSCYGKTKCTASNKNRGIIKTFSNGCDYVSNKGVDTVSVGNTLYYVNKQEGKSLYVKGEPIINFYDPLVFPSDEFDASISQVNEKINQSLAFIRKSDELL

SEQ ID NO: 22 - protein, 504 aa, synthetic construct
QNITEEFYQSTCSAVSKGYLSALRTGWYTSVITIELSNIKENKCNGTDAKVKLIKQELDKYKNAVTELQLLMQSTPAANSRARRELPRFMNYTLNNTKNTNVTLSKKRKRRFLGFLLGVGSAIASGIAVSKVLHLEGEVNKIKSALLSTNKAVVSLSNGVSVLTSKVLDLKNYIDKQLLPIVNKQSCSISNIETVIEFQQKNNRLLEITREFSVNAGVTTPVSTYMLTNSELLSLINDMPITNDQKKLMSSNVQIVRQQSYSIMSIIKEEVLAYVVQLPLYGVIDTPCWKLHTSPLCTTNTKEGSNICLTRTDRGWYCDNAGSVSFFPQAETCKVQSNRVFCDTMNSLTLPSEVNLCNIDIFNPKYDCKIMTSKTDVSSSVITSLGAIVSCYGKTKCTASNKNRGIIKTFSNGCDYVSNKGVDTVSVGNTLYYVNKQEGKSLYVKGEPIINFYDPLVFPSDEFDASISQVNEKINQSLAFIRKSDELLHNVNAGKSTTNIMITT

SEQ ID NO: 23 - protein, 488 aa, synthetic construct
QNITEEFYQSTCSAVSKGYLSALRTGWYTSVITIELSNIKENKCNGTDAKVKLIKQELDKYKNAVTELQLLMQSTPAANSQARRELPRFMNYTLNNTKNTNVTLSKKRKSSFLGFLLGVGSAIASGIAVSKVLHLEGEVNKIKSALLSTNKAVVSLSNGVSVLTSKVLDLKNYIDKQLLPIVNKQSCSISNIETVIEFQQKNNRLLEITREFSVNAGVTTPVSTYMLTNSELLSLINDMPITNDQKKLMSSNVQIVRQQSYSIMSIIKEEVLAYVVQLPLYGVIDTPCWKLHTSPLCTTNTKEGSNICLTRTDRGWYCDNAGSVSFFPQAETCKVQSNRVFCDTMNSLTLPSEVNLCNIDIFNPKYDCKIMTSKTDVSSSVITSLGAIVSCYGKTKCTASNKNRGIIKTFSNGCDYVSNKGVDTVSVGNTLYYVNKQEGKSLYVKGEPIINFYDPLVFPSDEFDASISQVNEKINQSLAFIRKSDELL

SEQ ID NO: 24 - protein, 84 aa, synthetic construct
QNITEEFYQSTCSAVSKGYLSALRTGWYTSVITIELSNIKENKCNGTDAKVKLIKQELDKYKNAVTELQLLMQSTPAANSRARR

SEQ ID NO: 25 - protein, 377 aa, synthetic construct
FLGFLLGVGSAIASGIAVSKVLHLEGEVNKIKSALLSTNKAVVSLSNGVSVLTSKVLDLKNYIDKQLLPIVNKQSCSISNIETVIEFQQKNNRLLEITREFSVNAGVTTPVSTYMLTNSELLSLINDMPITNDQKKLMSSNVQIVRQQSYSIMSIIKEEVLAYVVQLPLYGVIDTPCWKLHTSPLCTTNTKEGSNICLTRTDRGWYCDNAGSVSFFPQAETCKVQSNRVFCDTMNSLTLPSEVNLCNIDIFNPKYDCKIMTSKTDVSSSVITSLGAIVSCYGKTKCTASNKNRGIIKTFSNGCDYVSNKGVDTVSVGNTLYYVNKQEGKSLYVKGEPIINFYDPLVFPSDEFDASISQVNEKINQSLAFIRKSDELL

SEQ ID NO: 26 - protein, 466 aa, synthetic construct
QNITEEFYQSTCSAVSKGYLSALRTGWYTSVITIELSNIKENKCNGTDAKVKLIKQELDKYKNAVTELQLLMQSTPAANSQARGSGSGRSLGFLLGVGSAIASGIAVSKVLHLEGEVNKIKSALLSTNKAVVSLSNGVSVLTSKVLDLKNYIDKQLLPIVNKQSCSISNIETVIEFQQKNNRLLEITREFSVNAGVTTPVSTYMLTNSELLSLINDMPITNDQKKLMSSNVQIVRQQSYSIMSIIKEEVLAYVVQLPLYGVIDTPCWKLHTSPLCTTNTKEGSNICLTRTDRGWYCDNAGSVSFFPQAETCKVQSNRVFCDTMNSLTLPSEVNLCNIDIFNPKYDCKIMTSKTDVSSSVITSLGAIVSCYGKTKCTASNKNRGIIKTFSNGCDYVSNKGVDTVSVGNTLYYVNKQEGKSLYVKGEPIINFYDPLVFPSDEFDASISQVNEKINQSLAFIRKSDELL

SEQ ID NO: 27 - protein, 449 aa, synthetic construct
QNITEEFYQSTCSAVSKGYLSALRTGWYTSVITIELSNIKENKCNGTDAKVKLIKQELDKYKNAVTELQLLMQSTPAAGSGSAIASGIAVSKVLHLEGEVNKIKSALLSTNKAVVSLSNGVSVLTSKVLDLKNYIDKQLLPIVNKQSCSISNIETVIEFQQKNNRLLEITREFSVNAGVTTPVSTYMLTNSELLSLINDMPITNDQKKLMSSNVQIVRQQSYSIMSIIKEEVLAYVVQLPLYGVIDTPCWKLHTSPLCTTNTKEGSNICLTRTDRGWYCDNAGSVSFFPQAETCKVQSNRVFCDTMNSLTLPSEVNLCNIDIFNPKYDCKIMTSKTDVSSSVITSLGAIVSCYGKTKCTASNKNRGIIKTFSNGCDYVSNKGVDTVSVGNTLYYVNKQEGKSLYVKGEPIINFYDPLVFPSDEFDASISQVNEKINQSLAFIRKSDELL

SEQ ID NO: 28 - protein, 488 aa, synthetic construct
QNITEEFYQSTCSAVSRGYLSALRTGWYTSVITIELSNIKETKCNGTDTKVKLIKQELDKYKNAVTELQLLMQNTPAVNNRARREAPQYMNYTINTTKNLNVSISKKRKRRFLGFLLGVGSAIASGIAVSKVLHLEGEVNKIKNALQLTNKAVVSLSNGVSVLTSRVLDLKNYINNQLLPMVNRQSCRISNIETVIEFQQKNSRLLEITREFSVNAGVTTPLSTYMLTNSELLSLINDMPITNDQKKLMSSNVQIVRQQSYSIMSIIKEEVLAYVVQLPIYGVIDTPCWKLHTSPLCTTNIKEGSNICLTRTDRGWYCDNAGSVSFFPQADTCKVQSNRVFCDTMNSLTLPSEVSLCNTDIFNSKYDCKIMTSKTDISSSVITSLGAIVSCYGKTKCTASNKNRGIIKTFSNGCDYVSNKGVDTVSVGNTLYYVNKLEGKNLYVKGEPIINYYDPLVFPSDEFDASISQVNEKINQSLAFIRRSDELL

SEQ ID NO: 29 - protein, 504 aa, synthetic construct
QNITEEFYQSTCSAVSRGYLSALRTGWYTSVITIELSNIKETKCNGTDTKVKLIKQELDKYKNAVTELQLLMQNTPAVNNRARREAPQYMNYTINTTKNLNVSISKKRKRRFLGFLLGVGSAIASGIAVSKVLHLEGEVNKIKNALQLTNKAVVSLSNGVSVLTSRVLDLKNYINNQLLPMVNRQSCRISNIETVIEFQQKNSRLLEITREFSVNAGVTTPLSTYMLTNSELLSLINDMPITNDQKKLMSSNVQIVRQQSYSIMSIIKEEVLAYVVQLPIYGVIDTPCWKLHTSPLCTTNIKEGSNICLTRTDRGWYCDNAGSVSFFPQADTCKVQSNRVFCDTMNSLTLPSEVSLCNTDIFNSKYDCKIMTSKTDISSSVITSLGAIVSCYGKTKCTASNKNRGIIKTFSNGCDYVSNKGVDTVSVGNTLYYVNKLEGKNLYVKGEPIINYYDPLVFPSDEFDASISQVNEKINQSLAFIRRSDELLHNVNTGKSTTNIMITA

SEQ ID NO: 30 - protein, 488 aa, synthetic construct
QNITEEFYQSTCSAVSRGYLSALRTGWYTSVITIELSNIKETKCNGTDTKVKLIKQELDKYKNAVTELQLLMQNTPAVNNQARREAPQYMNYTINTTKNLNVSISKKRKSSFLGFLLGVGSAIASGIAVSKVLHLEGEVNKIKNALQLTNKAVVSLSNGVSVLTSRVLDLKNYINNQLLPMVNRQSCRISNIETVIEFQQKNSRLLEITREFSVNAGVTTPLSTYMLTNSELLSLINDMPITNDQKKLMSSNVQIVRQQSYSIMSIIKEEVLAYVVQLPIYGVIDTPCWKLHTSPLCTTNIKEGSNICLTRTDRGWYCDNAGSVSFFPQADTCKVQSNRVFCDTMNSLTLPSEVSLCNTDIFNSKYDCKIMTSKTDISSSVITSLGAIVSCYGKTKCTASNKNRGIIKTFSNGCDYVSNKGVDTVSVGNTLYYVNKLEGKNLYVKGEPIINYYDPLVFPSDEFDASISQVNEKINQSLAFIRRSDELL

SEQ ID NO: 31 - protein, 84 aa, synthetic construct
QNITEEFYQSTCSAVSRGYLSALRTGWYTSVITIELSNIKETKCNGTDTKVKLIKQELDKYKNAVTELQLLMQNTPAVNNRARR

SEQ ID NO: 32 - protein, 377 aa, synthetic construct
FLGFLLGVGSAIASGIAVSKVLHLEGEVNKIKNALQLTNKAVVSLSNGVSVLTSRVLDLKNYINNQLLPMVNRQSCRISNIETVIEFQQKNSRLLEITREFSVNAGVTTPLSTYMLTNSELLSLINDMPITNDQKKLMSSNVQIVRQQSYSIMSIIKEEVLAYVVQLPIYGVIDTPCWKLHTSPLCTTNIKEGSNICLTRTDRGWYCDNAGSVSFFPQADTCKVQSNRVFCDTMNSLTLPSEVSLCNTDIFNSKYDCKIMTSKTDISSSVITSLGAIVSCYGKTKCTASNKNRGIIKTFSNGCDYVSNKGVDTVSVGNTLYYVNKLEGKNLYVKGEPIINYYDPLVFPSDEFDASISQVNEKINQSLAFIRRSDELL

SEQ ID NO: 33 - protein, 466 aa, synthetic construct
QNITEEFYQSTCSAVSRGYLSALRTGWYTSVITIELSNIKETKCNGTDTKVKLIKQELDKYKNAVTELQLLMQNTPAVNNQARGSGSGRSLGFLLGVGSAIASGIAVSKVLHLEGEVNKIKNALQLTNKAVVSLSNGVSVLTSRVLDLKNYINNQLLPMVNRQSCRISNIETVIEFQQKNSRLLEITREFSVNAGVTTPLSTYMLTNSELLSLINDMPITNDQKKLMSSNVQIVRQQSYSIMSIIKEEVLAYVVQLPIYGVIDTPCWKLHTSPLCTTNIKEGSNICLTRTDRGWYCDNAGSVSFFPQADTCKVQSNRVFCDTMNSLTLPSEVSLCNTDIFNSKYDCKIMTSKTDISSSVITSLGAIVSCYGKTKCTASNKNRGIIKTFSNGCDYVSNKGVDTVSVGNTLYYVNKLEGKNLYVKGEPIINYYDPLVFPSDEFDASISQVNEKINQSLAFIRRSDELL

SEQ ID NO: 34 - protein, 449 aa, synthetic construct
QNITEEFYQSTCSAVSRGYLSALRTGWYTSVITIELSNIKETKCNGTDTKVKLIKQELDKYKNAVTELQLLMQNTPAVGSGSAIASGIAVSKVLHLEGEVNKIKNALQLTNKAVVSLSNGVSVLTSRVLDLKNYINNQLLPMVNRQSCRISNIETVIEFQQKNSRLLEITREFSVNAGVTTPLSTYMLTNSELLSLINDMPITNDQKKLMSSNVQIVRQQSYSIMSIIKEEVLAYVVQLPIYGVIDTPCWKLHTSPLCTTNIKEGSNICLTRTDRGWYCDNAGSVSFFPQADTCKVQSNRVFCDTMNSLTLPSEVSLCNTDIFNSKYDCKIMTSKTDISSSVITSLGAIVSCYGKTKCTASNKNRGIIKTFSNGCDYVSNKGVDTVSVGNTLYYVNKLEGKNLYVKGEPIINYYDPLVFPSDEFDASISQVNEKINQSLAFIRRSDELL

SEQ ID NO: 35 - protein, 466 aa, synthetic construct
QNITEEFYQSTCSAVSKGYLSALRTGWYTSVITIELSNIKENKCNGTDAKVKLIKQELDKYKNAVTELQLLMQSTPATNNQARGSGSGRSLGFLLGVGSAIASGVAVSKVLHLEGEVNKIKSALLSTNKAVVSLSNGVSVLTSKVLDLKNYIDKQLLPIVNKQSCSISNIETVIEFQQKMNRLLEITREFSVNAGVTTPVSTYMLTNSELLSLINDMPITNDQKKLMSNNVQIVRQQSYSIMSIIKEEVLAYVVQLPLYGVIDTPCWKLHTSPLCTTNTKEGSNICLTRTDRGWYCDNAGSVSFFPQAETCKVQSNRVFCDTMNSLTLPSEVNLCNVDIFNPKYDCKIMTSKTDVSSSVITSLGAIVSCYGKTKCTASNKNRGIIKTFSNGCDYVSNKGVDTVSVGNTLYYVNKQEGKSLYVKGEPIINFYDPLVFPSDEFDASISQVNEKINQSLAFIRKSDELL

SEQ ID NO: 36 - protein, 466 aa, synthetic construct
QNITEEFYQSTCSAVSKGYLSALRTGWYTSVITIELSNIKENKCNGTDAKVKLIKQELDKYKNAVTELQLLMQSTPATNNQARGSGSGRSLGFLLGVGSAIASGVAVSKVLHLEGEVNKIKSALLSTNKAVVSLSNGVSVLTSKVLDLKNYIDKQLLPIVNKQSCSISNIETVIEFQQKGNRLLEITREFSVNAGVTTPVSTYMLTNSELLSLINDMPITNDQKKLMSNNVQIVRQQSYSIMSIIKEEVLAYVVQLPLYGVIDTPCWKLHTSPLCTTNTKEGSNICLTRTDRGWYCDNAGSVSFFPQAETCKVQSNRVFCDTMNSLTLPSEVNLCNVDIFNPKYDCKIMTSKTDVSSSVITSLGAIVSCYGKTKCTASNKNRGIIKTFSNGCDYVSNKGVDTVSVGNTLYYVNKQEGKSLYVKGEPIINFYDPLVFPSDEFDASISQVNEKINQSLAFIRKSDELL

SEQ ID NO: 37 - protein, 466 aa, synthetic construct
QNITEEFYQSTCSAVSKGYLSALRTGWYTSVITIELSNIKENKCNGTDAKVKLIKQELDKYKNAVTELQLLMQSTPATNNQARGSGSGRSLGFLLGVGSAIASGVAVSKVLHLEGEVNKIKSALLSTNKAVVSLSNGVSVLTSKVLDLKNYIDKQLLPIVNKQSCSISNIETVIEFQQKANRLLEITREFSVNAGVTTPVSTYMLTNSELLSLINDMPITNDQKKLMSNNVQIVRQQSYSIMSIIKEEVLAYVVQLPLYGVIDTPCWKLHTSPLCTTNTKEGSNICLTRTDRGWYCDNAGSVSFFPQAETCKVQSNRVFCDTMNSLTLPSEVNLCNVDIFNPKYDCKIMTSKTDVSSSVITSLGAIVSCYGKTKCTASNKNRGIIKTFSNGCDYVSNKGVDTVSVGNTLYYVNKQEGKSLYVKGEPIINFYDPLVFPSDEFDASISQVNEKINQSLAFIRKSDELL

SEQ ID NO: 38 - protein, 466 aa, synthetic construct
QNITEEFYQSTCSAVSKGYLSALRTGWYTSVITIELSNIKENKCNGTDAKVKLIKQELDKYKNAVTELQLLMQSTPATNNQARGSGSGRSLGFLLGVGSAIASGVAVSKVLHLEGEVNKIKSALLSTNKAVVSLSNGVSVLTSKVLDLKNYIDKQLLPIVNKQSCSISNIETVIEFQQKVNRLLEITREFSVNAGVTTPVSTYMLTNSELLSLINDMPITNDQKKLMSNNVQIVRQQSYSIMSIIKEEVLAYVVQLPLYGVIDTPCWKLHTSPLCTTNTKEGSNICLTRTDRGWYCDNAGSVSFFPQAETCKVQSNRVFCDTMNSLTLPSEVNLCNVDIFNPKYDCKIMTSKTDVSSSVITSLGAIVSCYGKTKCTASNKNRGIIKTFSNGCDYVSNKGVDTVSVGNTLYYVNKQEGKSLYVKGEPIINFYDPLVFPSDEFDASISQVNEKINQSLAFIRKSDELL

SEQ ID NO: 39 - protein, 466 aa, synthetic construct
QNITEEFYQSTCSAVSKGYLSALRTGWYTSVITIELSNIKENKCNGTDAKVKLIKQELDKYKNAVTELQLLMQSTPATNNQARGSGSGRSLGFLLGVGSAIASGVAVSKVLHLEGEVNKIKSALLSTNKAVVSLSNGVSVLTSKVLDLKNYIDKQLLPIVNKQSCSISNIETVIEFQQKLNRLLEITREFSVNAGVTTPVSTYMLTNSELLSLINDMPITNDQKKLMSNNVQIVRQQSYSIMSIIKEEVLAYVVQLPLYGVIDTPCWKLHTSPLCTTNTKEGSNICLTRTDRGWYCDNAGSVSFFPQAETCKVQSNRVFCDTMNSLTLPSEVNLCNVDIFNPKYDCKIMTSKTDVSSSVITSLGAIVSCYGKTKCTASNKNRGIIKTFSNGCDYVSNKGVDTVSVGNTLYYVNKQEGKSLYVKGEPIINFYDPLVFPSDEFDASISQVNEKINQSLAFIRKSDELL

SEQ ID NO: 40 - protein, 466 aa, synthetic construct
QNITEEFYQSTCSAVSKGYLSALRTGWYTSVITIELSNIKENKCNGTDAKVKLIKQELDKYKNAVTELQLLMQSTPATNNQARGSGSGRSLGFLLGVGSAIASGVAVSKVLHLEGEVNKIKSALLSTNKAVVSLSNGVSVLTSKVLDLKNYIDKQLLPIVNKQSCSISNIETVIEFQQKINRLLEITREFSVNAGVTTPVSTYMLTNSELLSLINDMPITNDQKKLMSNNVQIVRQQSYSIMSIIKEEVLAYVVQLPLYGVIDTPCWKLHTSPLCTTNTKEGSNICLTRTDRGWYCDNAGSVSFFPQAETCKVQSNRVFCDTMNSLTLPSEVNLCNVDIFNPKYDCKIMTSKTDVSSSVITSLGAIVSCYGKTKCTASNKNRGIIKTFSNGCDYVSNKGVDTVSVGNTLYYVNKQEGKSLYVKGEPIINFYDPLVFPSDEFDASISQVNEKINQSLAFIRKSDELL

SEQ ID NO: 41 - protein, 466 aa, synthetic construct
QNITEEFYQSTCSAVSKGYLSALRTGWYTSVITIELSNIKENKCNGTDAKVKLIKQELDKYKNAVTELQLLMQSTPATNNQARGSGSGRSLGFLLGVGSAIASGVAVSKVLHLEGEVNKIKSALLSTNKAVVSLSNGVSVLTSKVLDLKNYIDKQLLPIVNKQSCSISNIETVIEFQQKWNRLLEITREFSVNAGVTTPVSTYMLTNSELLSLINDMPITNDQKKLMSNNVQIVRQQSYSIMSIIKEEVLAYVVQLPLYGVIDTPCWKLHTSPLCTTNTKEGSNICLTRTDRGWYCDNAGSVSFFPQAETCKVQSNRVFCDTMNSLTLPSEVNLCNVDIFNPKYDCKIMTSKTDVSSSVITSLGAIVSCYGKTKCTASNKNRGIIKTFSNGCDYVSNKGVDTVSVGNTLYYVNKQEGKSLYVKGEPIINFYDPLVFPSDEFDASISQVNEKINQSLAFIRKSDELL

SEQ ID NO: 42 - protein, 466 aa, synthetic construct
QNITEEFYQSTCSAVSKGYLSALRTGWYTSVITIELSNIKENKCNGTDAKVKLIKQELDKYKNAVTELQLLMQSTPATNNQARGSGSGRSLGFLLGVGSAIASGVAVSKVLHLEGEVNKIKSALLSTNKAVVSLSNGVSVLTSKVLDLKNYIDKQLLPIVNKQSCSISNIETVIEFQQKFNRLLEITREFSVNAGVTTPVSTYMLTNSELLSLINDMPITNDQKKLMSNNVQIVRQQSYSIMSIIKEEVLAYVVQLPLYGVIDTPCWKLHTSPLCTTNTKEGSNICLTRTDRGWYCDNAGSVSFFPQAETCKVQSNRVFCDTMNSLTLPSEVNLCNVDIFNPKYDCKIMTSKTDVSSSVITSLGAIVSCYGKTKCTASNKNRGIIKTFSNGCDYVSNKGVDTVSVGNTLYYVNKQEGKSLYVKGEPIINFYDPLVFPSDEFDASISQVNEKINQSLAFIRKSDELL

SEQ ID NO: 43 - protein, 466 aa, synthetic construct
QNITEEFYQSTCSAVSKGYLSALRTGWYTSVITIELSNIKENKCNGTDAKVKLIKQELDKYKNAVTELQLLMQSTPATNNQARGSGSGRSLGFLLGVGSAIASGVAVSKVLHLEGEVNKIKSALLSTNKAVVSLSNGVSVLTSKVLDLKNYIDKQLLPIVNKQSCSISNIETVIEFQQKPNRLLEITREFSVNAGVTTPVSTYMLTNSELLSLINDMPITNDQKKLMSNNVQIVRQQSYSIMSIIKEEVLAYVVQLPLYGVIDTPCWKLHTSPLCTTNTKEGSNICLTRTDRGWYCDNAGSVSFFPQAETCKVQSNRVFCDTMNSLTLPSEVNLCNVDIFNPKYDCKIMTSKTDVSSSVITSLGAIVSCYGKTKCTASNKNRGIIKTFSNGCDYVSNKGVDTVSVGNTLYYVNKQEGKSLYVKGEPIINFYDPLVFPSDEFDASISQVNEKINQSLAFIRKSDELL

SEQ ID NO: 44 - protein, 466 aa, synthetic construct
QNITEEFYQSTCSAVSKGYLSALRTGWYTSVITIELSNIKENKCNGTDAKVKLIKQELDKYKNAVTELQLLMQSTPATNNQARGSGSGRSLGFLLGVGSAIASGVAVSKVLHLEGEVNKIKSALLSTNKAVVSLSNGVSVLTSKVLDLKNYIDKQLLPIVNKQSCSISNIETVIEFQQKSNRLLEITREFSVNAGVTTPVSTYMLTNSELLSLINDMPITNDQKKLMSNNVQIVRQQSYSIMSIIKEEVLAYVVQLPLYGVIDTPCWKLHTSPLCTTNTKEGSNICLTRTDRGWYCDNAGSVSFFPQAETCKVQSNRVFCDTMNSLTLPSEVNLCNVDIFNPKYDCKIMTSKTDVSSSVITSLGAIVSCYGKTKCTASNKNRGIIKTFSNGCDYVSNKGVDTVSVGNTLYYVNKQEGKSLYVKGEPIINFYDPLVFPSDEFDASISQVNEKINQSLAFIRKSDELL

SEQ ID NO: 45 - protein, 466 aa, synthetic construct
QNITEEFYQSTCSAVSKGYLSALRTGWYTSVITIELSNIKENKCNGTDAKVKLIKQELDKYKNAVTELQLLMQSTPATNNQARGSGSGRSLGFLLGVGSAIASGVAVSKVLHLEGEVNKIKSALLSTNKAVVSLSNGVSVLTSKVLDLKNYIDKQLLPIVNKQSCSISNIETVIEFQQKTNRLLEITREFSVNAGVTTPVSTYMLTNSELLSLINDMPITNDQKKLMSNNVQIVRQQSYSIMSIIKEEVLAYVVQLPLYGVIDTPCWKLHTSPLCTTNTKEGSNICLTRTDRGWYCDNAGSVSFFPQAETCKVQSNRVFCDTMNSLTLPSEVNLCNVDIFNPKYDCKIMTSKTDVSSSVITSLGAIVSCYGKTKCTASNKNRGIIKTFSNGCDYVSNKGVDTVSVGNTLYYVNKQEGKSLYVKGEPIINFYDPLVFPSDEFDASISQVNEKINQSLAFIRKSDELL

SEQ ID NO: 46 - protein, 466 aa, synthetic construct
QNITEEFYQSTCSAVSKGYLSALRTGWYTSVITIELSNIKENKCNGTDAKVKLIKQELDKYKNAVTELQLLMQSTPATNNQARGSGSGRSLGFLLGVGSAIASGVAVSKVLHLEGEVNKIKSALLSTNKAVVSLSNGVSVLTSKVLDLKNYIDKQLLPIVNKQSCSISNIETVIEFQQKCNRLLEITREFSVNAGVTTPVSTYMLTNSELLSLINDMPITNDQKKLMSNNVQIVRQQSYSIMSIIKEEVLAYVVQLPLYGVIDTPCWKLHTSPLCTTNTKEGSNICLTRTDRGWYCDNAGSVSFFPQAETCKVQSNRVFCDTMNSLTLPSEVNLCNVDIFNPKYDCKIMTSKTDVSSSVITSLGAIVSCYGKTKCTASNKNRGIIKTFSNGCDYVSNKGVDTVSVGNTLYYVNKQEGKSLYVKGEPIINFYDPLVFPSDEFDASISQVNEKINQSLAFIRKSDELL

SEQ ID NO: 47 - protein, 466 aa, synthetic construct
QNITEEFYQSTCSAVSKGYLSALRTGWYTSVITIELSNIKENKCNGTDAKVKLIKQELDKYKNAVTELQLLMQSTPATNNQARGSGSGRSLGFLLGVGSAIASGVAVSKVLHLEGEVNKIKSALLSTNKAVVSLSNGVSVLTSKVLDLKNYIDKQLLPIVNKQSCSISNIETVIEFQQKYNRLLEITREFSVNAGVTTPVSTYMLTNSELLSLINDMPITNDQKKLMSNNVQIVRQQSYSIMSIIKEEVLAYVVQLPLYGVIDTPCWKLHTSPLCTTNTKEGSNICLTRTDRGWYCDNAGSVSFFPQAETCKVQSNRVFCDTMNSLTLPSEVNLCNVDIFNPKYDCKIMTSKTDVSSSVITSLGAIVSCYGKTKCTASNKNRGIIKTFSNGCDYVSNKGVDTVSVGNTLYYVNKQEGKSLYVKGEPIINFYDPLVFPSDEFDASISQVNEKINQSLAFIRKSDELL

SEQ ID NO: 48 - protein, 466 aa, synthetic construct
QNITEEFYQSTCSAVSKGYLSALRTGWYTSVITIELSNIKENKCNGTDAKVKLIKQELDKYKNAVTELQLLMQSTPATNNQARGSGSGRSLGFLLGVGSAIASGVAVSKVLHLEGEVNKIKSALLSTNKAVVSLSNGVSVLTSKVLDLKNYIDKQLLPIVNKQSCSISNIETVIEFQQKQNRLLEITREFSVNAGVTTPVSTYMLTNSELLSLINDMPITNDQKKLMSNNVQIVRQQSYSIMSIIKEEVLAYVVQLPLYGVIDTPCWKLHTSPLCTTNTKEGSNICLTRTDRGWYCDNAGSVSFFPQAETCKVQSNRVFCDTMNSLTLPSEVNLCNVDIFNPKYDCKIMTSKTDVSSSVITSLGAIVSCYGKTKCTASNKNRGIIKTFSNGCDYVSNKGVDTVSVGNTLYYVNKQEGKSLYVKGEPIINFYDPLVFPSDEFDASISQVNEKINQSLAFIRKSDELL

SEQ ID NO: 49 - protein, 466 aa, synthetic construct
QNITEEFYQSTCSAVSKGYLSALRTGWYTSVITIELSNIKENKCNGTDAKVKLIKQELDKYKNAVTELQLLMQSTPATNNQARGSGSGRSLGFLLGVGSAIASGVAVSKVLHLEGEVNKIKSALLSTNKAVVSLSNGVSVLTSKVLDLKNYIDKQLLPIVNKQSCSISNIETVIEFQQKDNRLLEITREFSVNAGVTTPVSTYMLTNSELLSLINDMPITNDQKKLMSNNVQIVRQQSYSIMSIIKEEVLAYVVQLPLYGVIDTPCWKLHTSPLCTTNTKEGSNICLTRTDRGWYCDNAGSVSFFPQAETCKVQSNRVFCDTMNSLTLPSEVNLCNVDIFNPKYDCKIMTSKTDVSSSVITSLGAIVSCYGKTKCTASNKNRGIIKTFSNGCDYVSNKGVDTVSVGNTLYYVNKQEGKSLYVKGEPIINFYDPLVFPSDEFDASISQVNEKINQSLAFIRKSDELL

SEQ ID NO: 50 - protein, 466 aa, synthetic construct
QNITEEFYQSTCSAVSKGYLSALRTGWYTSVITIELSNIKENKCNGTDAKVKLIKQELDKYKNAVTELQLLMQSTPATNNQARGSGSGRSLGFLLGVGSAIASGVAVSKVLHLEGEVNKIKSALLSTNKAVVSLSNGVSVLTSKVLDLKNYIDKQLLPIVNKQSCSISNIETVIEFQQKENRLLEITREFSVNAGVTTPVSTYMLTNSELLSLINDMPITNDQKKLMSNNVQIVRQQSYSIMSIIKEEVLAYVVQLPLYGVIDTPCWKLHTSPLCTTNTKEGSNICLTRTDRGWYCDNAGSVSFFPQAETCKVQSNRVFCDTMNSLTLPSEVNLCNVDIFNPKYDCKIMTSKTDVSSSVITSLGAIVSCYGKTKCTASNKNRGIIKTFSNGCDYVSNKGVDTVSVGNTLYYVNKQEGKSLYVKGEPIINFYDPLVFPSDEFDASISQVNEKINQSLAFIRKSDELL

SEQ ID NO: 51 - protein, 466 aa, synthetic construct
QNITEEFYQSTCSAVSKGYLSALRTGWYTSVITIELSNIKENKCNGTDAKVKLIKQELDKYKNAVTELQLLMQSTPATNNQARGSGSGRSLGFLLGVGSAIASGVAVSKVLHLEGEVNKIKSALLSTNKAVVSLSNGVSVLTSKVLDLKNYIDKQLLPIVNKQSCSISNIETVIEFQQKKNRLLEITREFSVNAGVTTPVSTYMLTNSELLSLINDMPITNDQKKLMSNNVQIVRQQSYSIMSIIKEEVLAYVVQLPLYGVIDTPCWKLHTSPLCTTNTKEGSNICLTRTDRGWYCDNAGSVSFFPQAETCKVQSNRVFCDTMNSLTLPSEVNLCNVDIFNPKYDCKIMTSKTDVSSSVITSLGAIVSCYGKTKCTASNKNRGIIKTFSNGCDYVSNKGVDTVSVGNTLYYVNKQEGKSLYVKGEPIINFYDPLVFPSDEFDASISQVNEKINQSLAFIRKSDELL

SEQ ID NO: 52 - protein, 466 aa, synthetic construct
QNITEEFYQSTCSAVSKGYLSALRTGWYTSVITIELSNIKENKCNGTDAKVKLIKQELDKYKNAVTELQLLMQSTPATNNQARGSGSGRSLGFLLGVGSAIASGVAVSKVLHLEGEVNKIKSALLSTNKAVVSLSNGVSVLTSKVLDLKNYIDKQLLPIVNKQSCSISNIETVIEFQQKRNRLLEITREFSVNAGVTTPVSTYMLTNSELLSLINDMPITNDQKKLMSNNVQIVRQQSYSIMSIIKEEVLAYVVQLPLYGVIDTPCWKLHTSPLCTTNTKEGSNICLTRTDRGWYCDNAGSVSFFPQAETCKVQSNRVFCDTMNSLTLPSEVNLCNVDIFNPKYDCKIMTSKTDVSSSVITSLGAIVSCYGKTKCTASNKNRGIIKTFSNGCDYVSNKGVDTVSVGNTLYYVNKQEGKSLYVKGEPIINFYDPLVFPSDEFDASISQVNEKINQSLAFIRKSDELL

SEQ ID NO: 53 - protein, 466 aa, synthetic construct
QNITEEFYQSTCSAVSKGYLSALRTGWYTSVITIELSNIKENKCNGTDAKVKLIKQELDKYKNAVTELQLLMQSTPATNNQARGSGSGRSLGFLLGVGSAIASGVAVSKVLHLEGEVNKIKSALLSTNKAVVSLSNGVSVLTSKVLDLKNYIDKQLLPIVNKQSCSISNIETVIEFQQKHNRLLEITREFSVNAGVTTPVSTYMLTNSELLSLINDMPITNDQKKLMSNNVQIVRQQSYSIMSIIKEEVLAYVVQLPLYGVIDTPCWKLHTSPLCTTNTKEGSNICLTRTDRGWYCDNAGSVSFFPQAETCKVQSNRVFCDTMNSLTLPSEVNLCNVDIFNPKYDCKIMTSKTDVSSSVITSLGAIVSCYGKTKCTASNKNRGIIKTFSNGCDYVSNKGVDTVSVGNTLYYVNKQEGKSLYVKGEPIINFYDPLVFPSDEFDASISQVNEKINQSLAFIRKSDELL

SEQ ID NO: 54 - protein, 466 aa, synthetic construct
QNITEEFYQSTCSAVSKGYLSALRTGWYTSVITIELSNIKENKCNGTDAKVKLIKQELDKYKNAVTELQLLMQSTPATNNQARGSGSGRSLGFLLGVGSAIASGVAVSKVLHLEGEVNKIKSALLSTNKAVVSLSNGVSVLTSKVLDLKNYIDKQLLPIVNKQSCSISNIETVIEFQQKNNRMLEITREFSVNAGVTTPVSTYMLTNSELLSLINDMPITNDQKKLMSNNVQIVRQQSYSIMSIIKEEVLAYVVQLPLYGVIDTPCWKLHTSPLCTTNTKEGSNICLTRTDRGWYCDNAGSVSFFPQAETCKVQSNRVFCDTMNSLTLPSEVNLCNVDIFNPKYDCKIMTSKTDVSSSVITSLGAIVSCYGKTKCTASNKNRGIIKTFSNGCDYVSNKGVDTVSVGNTLYYVNKQEGKSLYVKGEPIINFYDPLVFPSDEFDASISQVNEKINQSLAFIRKSDELL

SEQ ID NO: 55 - protein, 466 aa, synthetic construct
QNITEEFYQSTCSAVSKGYLSALRTGWYTSVITIELSNIKENKCNGTDAKVKLIKQELDKYKNAVTELQLLMQSTPATNNQARGSGSGRSLGFLLGVGSAIASGVAVSKVLHLEGEVNKIKSALLSTNKAVVSLSNGVSVLTSKVLDLKNYIDKQLLPIVNKQSCSISNIETVIEFQQKNNRGLEITREFSVNAGVTTPVSTYMLTNSELLSLINDMPITNDQKKLMSNNVQIVRQQSYSIMSIIKEEVLAYVVQLPLYGVIDTPCWKLHTSPLCTTNTKEGSNICLTRTDRGWYCDNAGSVSFFPQAETCKVQSNRVFCDTMNSLTLPSEVNLCNVDIFNPKYDCKIMTSKTDVSSSVITSLGAIVSCYGKTKCTASNKNRGIIKTFSNGCDYVSNKGVDTVSVGNTLYYVNKQEGKSLYVKGEPIINFYDPLVFPSDEFDASISQVNEKINQSLAFIRKSDELL

SEQ ID NO: 56 - protein, 466 aa, synthetic construct
QNITEEFYQSTCSAVSKGYLSALRTGWYTSVITIELSNIKENKCNGTDAKVKLIKQELDKYKNAVTELQLLMQSTPATNNQARGSGSGRSLGFLLGVGSAIASGVAVSKVLHLEGEVNKIKSALLSTNKAVVSLSNGVSVLTSKVLDLKNYIDKQLLPIVNKQSCSISNIETVIEFQQKNNRALEITREFSVNAGVTTPVSTYMLTNSELLSLINDMPITNDQKKLMSNNVQIVRQQSYSIMSIIKEEVLAYVVQLPLYGVIDTPCWKLHTSPLCTTNTKEGSNICLTRTDRGWYCDNAGSVSFFPQAETCKVQSNRVFCDTMNSLTLPSEVNLCNVDIFNPKYDCKIMTSKTDVSSSVITSLGAIVSCYGKTKCTASNKNRGIIKTFSNGCDYVSNKGVDTVSVGNTLYYVNKQEGKSLYVKGEPIINFYDPLVFPSDEFDASISQVNEKINQSLAFIRKSDELL

SEQ ID NO: 57 - protein, 466 aa, synthetic construct
QNITEEFYQSTCSAVSKGYLSALRTGWYTSVITIELSNIKENKCNGTDAKVKLIKQELDKYKNAVTELQLLMQSTPATNNQARGSGSGRSLGFLLGVGSAIASGVAVSKVLHLEGEVNKIKSALLSTNKAVVSLSNGVSVLTSKVLDLKNYIDKQLLPIVNKQSCSISNIETVIEFQQKNNRVLEITREFSVNAGVTTPVSTYMLTNSELLSLINDMPITNDQKKLMSNNVQIVRQQSYSIMSIIKEEVLAYVVQLPLYGVIDTPCWKLHTSPLCTTNTKEGSNICLTRTDRGWYCDNAGSVSFFPQAETCKVQSNRVFCDTMNSLTLPSEVNLCNVDIFNPKYDCKIMTSKTDVSSSVITSLGAIVSCYGKTKCTASNKNRGIIKTFSNGCDYVSNKGVDTVSVGNTLYYVNKQEGKSLYVKGEPIINFYDPLVFPSDEFDASISQVNEKINQSLAFIRKSDELL

SEQ ID NO: 58 - protein, 466 aa, synthetic construct
QNITEEFYQSTCSAVSKGYLSALRTGWYTSVITIELSNIKENKCNGTDAKVKLIKQELDKYKNAVTELQLLMQSTPATNNQARGSGSGRSLGFLLGVGSAIASGVAVSKVLHLEGEVNKIKSALLSTNKAVVSLSNGVSVLTSKVLDLKNYIDKQLLPIVNKQSCSISNIETVIEFQQKNNRILEITREFSVNAGVTTPVSTYMLTNSELLSLINDMPITNDQKKLMSNNVQIVRQQSYSIMSIIKEEVLAYVVQLPLYGVIDTPCWKLHTSPLCTTNTKEGSNICLTRTDRGWYCDNAGSVSFFPQAETCKVQSNRVFCDTMNSLTLPSEVNLCNVDIFNPKYDCKIMTSKTDVSSSVITSLGAIVSCYGKTKCTASNKNRGIIKTFSNGCDYVSNKGVDTVSVGNTLYYVNKQEGKSLYVKGEPIINFYDPLVFPSDEFDASISQVNEKINQSLAFIRKSDELL

SEQ ID NO: 59 - protein, 466 aa, synthetic construct
QNITEEFYQSTCSAVSKGYLSALRTGWYTSVITIELSNIKENKCNGTDAKVKLIKQELDKYKNAVTELQLLMQSTPATNNQARGSGSGRSLGFLLGVGSAIASGVAVSKVLHLEGEVNKIKSALLSTNKAVVSLSNGVSVLTSKVLDLKNYIDKQLLPIVNKQSCSISNIETVIEFQQKNNRWLEITREFSVNAGVTTPVSTYMLTNSELLSLINDMPITNDQKKLMSNNVQIVRQQSYSIMSIIKEEVLAYVVQLPLYGVIDTPCWKLHTSPLCTTNTKEGSNICLTRTDRGWYCDNAGSVSFFPQAETCKVQSNRVFCDTMNSLTLPSEVNLCNVDIFNPKYDCKIMTSKTDVSSSVITSLGAIVSCYGKTKCTASNKNRGIIKTFSNGCDYVSNKGVDTVSVGNTLYYVNKQEGKSLYVKGEPIINFYDPLVFPSDEFDASISQVNEKINQSLAFIRKSDELL

SEQ ID NO: 60 - protein, 466 aa, synthetic construct
QNITEEFYQSTCSAVSKGYLSALRTGWYTSVITIELSNIKENKCNGTDAKVKLIKQELDKYKNAVTELQLLMQSTPATNNQARGSGSGRSLGFLLGVGSAIASGVAVSKVLHLEGEVNKIKSALLSTNKAVVSLSNGVSVLTSKVLDLKNYIDKQLLPIVNKQSCSISNIETVIEFQQKNNRFLEITREFSVNAGVTTPVSTYMLTNSELLSLINDMPITNDQKKLMSNNVQIVRQQSYSIMSIIKEEVLAYVVQLPLYGVIDTPCWKLHTSPLCTTNTKEGSNICLTRTDRGWYCDNAGSVSFFPQAETCKVQSNRVFCDTMNSLTLPSEVNLCNVDIFNPKYDCKIMTSKTDVSSSVITSLGAIVSCYGKTKCTASNKNRGIIKTFSNGCDYVSNKGVDTVSVGNTLYYVNKQEGKSLYVKGEPIINFYDPLVFPSDEFDASISQVNEKINQSLAFIRKSDELL

SEQ ID NO: 61 - protein, 466 aa, synthetic construct
QNITEEFYQSTCSAVSKGYLSALRTGWYTSVITIELSNIKENKCNGTDAKVKLIKQELDKYKNAVTELQLLMQSTPATNNQARGSGSGRSLGFLLGVGSAIASGVAVSKVLHLEGEVNKIKSALLSTNKAVVSLSNGVSVLTSKVLDLKNYIDKQLLPIVNKQSCSISNIETVIEFQQKNNRPLEITREFSVNAGVTTPVSTYMLTNSELLSLINDMPITNDQKKLMSNNVQIVRQQSYSIMSIIKEEVLAYVVQLPLYGVIDTPCWKLHTSPLCTTNTKEGSNICLTRTDRGWYCDNAGSVSFFPQAETCKVQSNRVFCDTMNSLTLPSEVNLCNVDIFNPKYDCKIMTSKTDVSSSVITSLGAIVSCYGKTKCTASNKNRGIIKTFSNGCDYVSNKGVDTVSVGNTLYYVNKQEGKSLYVKGEPIINFYDPLVFPSDEFDASISQVNEKINQSLAFIRKSDELL

SEQ ID NO: 62 - protein, 466 aa, synthetic construct
QNITEEFYQSTCSAVSKGYLSALRTGWYTSVITIELSNIKENKCNGTDAKVKLIKQELDKYKNAVTELQLLMQSTPATNNQARGSGSGRSLGFLLGVGSAIASGVAVSKVLHLEGEVNKIKSALLSTNKAVVSLSNGVSVLTSKVLDLKNYIDKQLLPIVNKQSCSISNIETVIEFQQKNNRSLEITREFSVNAGVTTPVSTYMLTNSELLSLINDMPITNDQKKLMSNNVQIVRQQSYSIMSIIKEEVLAYVVQLPLYGVIDTPCWKLHTSPLCTTNTKEGSNICLTRTDRGWYCDNAGSVSFFPQAETCKVQSNRVFCDTMNSLTLPSEVNLCNVDIFNPKYDCKIMTSKTDVSSSVITSLGAIVSCYGKTKCTASNKNRGIIKTFSNGCDYVSNKGVDTVSVGNTLYYVNKQEGKSLYVKGEPIINFYDPLVFPSDEFDASISQVNEKINQSLAFIRKSDELL

SEQ ID NO: 63 - protein, 466 aa, synthetic construct
QNITEEFYQSTCSAVSKGYLSALRTGWYTSVITIELSNIKENKCNGTDAKVKLIKQELDKYKNAVTELQLLMQSTPATNNQARGSGSGRSLGFLLGVGSAIASGVAVSKVLHLEGEVNKIKSALLSTNKAVVSLSNGVSVLTSKVLDLKNYIDKQLLPIVNKQSCSISNIETVIEFQQKNNRTLEITREFSVNAGVTTPVSTYMLTNSELLSLINDMPITNDQKKLMSNNVQIVRQQSYSIMSIIKEEVLAYVVQLPLYGVIDTPCWKLHTSPLCTTNTKEGSNICLTRTDRGWYCDNAGSVSFFPQAETCKVQSNRVFCDTMNSLTLPSEVNLCNVDIFNPKYDCKIMTSKTDVSSSVITSLGAIVSCYGKTKCTASNKNRGIIKTFSNGCDYVSNKGVDTVSVGNTLYYVNKQEGKSLYVKGEPIINFYDPLVFPSDEFDASISQVNEKINQSLAFIRKSDELL

SEQ ID NO: 64 - protein, 466 aa, synthetic construct
QNITEEFYQSTCSAVSKGYLSALRTGWYTSVITIELSNIKENKCNGTDAKVKLIKQELDKYKNAVTELQLLMQSTPATNNQARGSGSGRSLGFLLGVGSAIASGVAVSKVLHLEGEVNKIKSALLSTNKAVVSLSNGVSVLTSKVLDLKNYIDKQLLPIVNKQSCSISNIETVIEFQQKNNRCLEITREFSVNAGVTTPVSTYMLTNSELLSLINDMPITNDQKKLMSNNVQIVRQQSYSIMSIIKEEVLAYVVQLPLYGVIDTPCWKLHTSPLCTTNTKEGSNICLTRTDRGWYCDNAGSVSFFPQAETCKVQSNRVFCDTMNSLTLPSEVNLCNVDIFNPKYDCKIMTSKTDVSSSVITSLGAIVSCYGKTKCTASNKNRGIIKTFSNGCDYVSNKGVDTVSVGNTLYYVNKQEGKSLYVKGEPIINFYDPLVFPSDEFDASISQVNEKINQSLAFIRKSDELL

SEQ ID NO: 65 - protein, 466 aa, synthetic construct
QNITEEFYQSTCSAVSKGYLSALRTGWYTSVITIELSNIKENKCNGTDAKVKLIKQELDKYKNAVTELQLLMQSTPATNNQARGSGSGRSLGFLLGVGSAIASGVAVSKVLHLEGEVNKIKSALLSTNKAVVSLSNGVSVLTSKVLDLKNYIDKQLLPIVNKQSCSISNIETVIEFQQKNNRYLEITREFSVNAGVTTPVSTYMLTNSELLSLINDMPITNDQKKLMSNNVQIVRQQSYSIMSIIKEEVLAYVVQLPLYGVIDTPCWKLHTSPLCTTNTKEGSNICLTRTDRGWYCDNAGSVSFFPQAETCKVQSNRVFCDTMNSLTLPSEVNLCNVDIFNPKYDCKIMTSKTDVSSSVITSLGAIVSCYGKTKCTASNKNRGIIKTFSNGCDYVSNKGVDTVSVGNTLYYVNKQEGKSLYVKGEPIINFYDPLVFPSDEFDASISQVNEKINQSLAFIRKSDELL

SEQ ID NO: 66 - protein, 466 aa, synthetic construct
QNITEEFYQSTCSAVSKGYLSALRTGWYTSVITIELSNIKENKCNGTDAKVKLIKQELDKYKNAVTELQLLMQSTPATNNQARGSGSGRSLGFLLGVGSAIASGVAVSKVLHLEGEVNKIKSALLSTNKAVVSLSNGVSVLTSKVLDLKNYIDKQLLPIVNKQSCSISNIETVIEFQQKNNRQLEITREFSVNAGVTTPVSTYMLTNSELLSLINDMPITNDQKKLMSNNVQIVRQQSYSIMSIIKEEVLAYVVQLPLYGVIDTPCWKLHTSPLCTTNTKEGSNICLTRTDRGWYCDNAGSVSFFPQAETCKVQSNRVFCDTMNSLTLPSEVNLCNVDIFNPKYDCKIMTSKTDVSSSVITSLGAIVSCYGKTKCTASNKNRGIIKTFSNGCDYVSNKGVDTVSVGNTLYYVNKQEGKSLYVKGEPIINFYDPLVFPSDEFDASISQVNEKINQSLAFIRKSDELL

SEQ ID NO: 67 - protein, 466 aa, synthetic construct
QNITEEFYQSTCSAVSKGYLSALRTGWYTSVITIELSNIKENKCNGTDAKVKLIKQELDKYKNAVTELQLLMQSTPATNNQARGSGSGRSLGFLLGVGSAIASGVAVSKVLHLEGEVNKIKSALLSTNKAVVSLSNGVSVLTSKVLDLKNYIDKQLLPIVNKQSCSISNIETVIEFQQKNNRNLEITREFSVNAGVTTPVSTYMLTNSELLSLINDMPITNDQKKLMSNNVQIVRQQSYSIMSIIKEEVLAYVVQLPLYGVIDTPCWKLHTSPLCTTNTKEGSNICLTRTDRGWYCDNAGSVSFFPQAETCKVQSNRVFCDTMNSLTLPSEVNLCNVDIFNPKYDCKIMTSKTDVSSSVITSLGAIVSCYGKTKCTASNKNRGIIKTFSNGCDYVSNKGVDTVSVGNTLYYVNKQEGKSLYVKGEPIINFYDPLVFPSDEFDASISQVNEKINQSLAFIRKSDELL

SEQ ID NO: 68 - protein, 466 aa, synthetic construct
QNITEEFYQSTCSAVSKGYLSALRTGWYTSVITIELSNIKENKCNGTDAKVKLIKQELDKYKNAVTELQLLMQSTPATNNQARGSGSGRSLGFLLGVGSAIASGVAVSKVLHLEGEVNKIKSALLSTNKAVVSLSNGVSVLTSKVLDLKNYIDKQLLPIVNKQSCSISNIETVIEFQQKNNRDLEITREFSVNAGVTTPVSTYMLTNSELLSLINDMPITNDQKKLMSNNVQIVRQQSYSIMSIIKEEVLAYVVQLPLYGVIDTPCWKLHTSPLCTTNTKEGSNICLTRTDRGWYCDNAGSVSFFPQAETCKVQSNRVFCDTMNSLTLPSEVNLCNVDIFNPKYDCKIMTSKTDVSSSVITSLGAIVSCYGKTKCTASNKNRGIIKTFSNGCDYVSNKGVDTVSVGNTLYYVNKQEGKSLYVKGEPIINFYDPLVFPSDEFDASISQVNEKINQSLAFIRKSDELL

SEQ ID NO: 69 - protein, 466 aa, synthetic construct
QNITEEFYQSTCSAVSKGYLSALRTGWYTSVITIELSNIKENKCNGTDAKVKLIKQELDKYKNAVTELQLLMQSTPATNNQARGSGSGRSLGFLLGVGSAIASGVAVSKVLHLEGEVNKIKSALLSTNKAVVSLSNGVSVLTSKVLDLKNYIDKQLLPIVNKQSCSISNIETVIEFQQKNNRELEITREFSVNAGVTTPVSTYMLTNSELLSLINDMPITNDQKKLMSNNVQIVRQQSYSIMSIIKEEVLAYVVQLPLYGVIDTPCWKLHTSPLCTTNTKEGSNICLTRTDRGWYCDNAGSVSFFPQAETCKVQSNRVFCDTMNSLTLPSEVNLCNVDIFNPKYDCKIMTSKTDVSSSVITSLGAIVSCYGKTKCTASNKNRGIIKTFSNGCDYVSNKGVDTVSVGNTLYYVNKQEGKSLYVKGEPIINFYDPLVFPSDEFDASISQVNEKINQSLAFIRKSDELL

SEQ ID NO: 70 - protein, 466 aa, synthetic construct
QNITEEFYQSTCSAVSKGYLSALRTGWYTSVITIELSNIKENKCNGTDAKVKLIKQELDKYKNAVTELQLLMQSTPATNNQARGSGSGRSLGFLLGVGSAIASGVAVSKVLHLEGEVNKIKSALLSTNKAVVSLSNGVSVLTSKVLDLKNYIDKQLLPIVNKQSCSISNIETVIEFQQKNNRKLEITREFSVNAGVTTPVSTYMLTNSELLSLINDMPITNDQKKLMSNNVQIVRQQSYSIMSIIKEEVLAYVVQLPLYGVIDTPCWKLHTSPLCTTNTKEGSNICLTRTDRGWYCDNAGSVSFFPQAETCKVQSNRVFCDTMNSLTLPSEVNLCNVDIFNPKYDCKIMTSKTDVSSSVITSLGAIVSCYGKTKCTASNKNRGIIKTFSNGCDYVSNKGVDTVSVGNTLYYVNKQEGKSLYVKGEPIINFYDPLVFPSDEFDASISQVNEKINQSLAFIRKSDELL

SEQ ID NO: 71 - protein, 466 aa, synthetic construct
QNITEEFYQSTCSAVSKGYLSALRTGWYTSVITIELSNIKENKCNGTDAKVKLIKQELDKYKNAVTELQLLMQSTPATNNQARGSGSGRSLGFLLGVGSAIASGVAVSKVLHLEGEVNKIKSALLSTNKAVVSLSNGVSVLTSKVLDLKNYIDKQLLPIVNKQSCSISNIETVIEFQQKNNRRLEITREFSVNAGVTTPVSTYMLTNSELLSLINDMPITNDQKKLMSNNVQIVRQQSYSIMSIIKEEVLAYVVQLPLYGVIDTPCWKLHTSPLCTTNTKEGSNICLTRTDRGWYCDNAGSVSFFPQAETCKVQSNRVFCDTMNSLTLPSEVNLCNVDIFNPKYDCKIMTSKTDVSSSVITSLGAIVSCYGKTKCTASNKNRGIIKTFSNGCDYVSNKGVDTVSVGNTLYYVNKQEGKSLYVKGEPIINFYDPLVFPSDEFDASISQVNEKINQSLAFIRKSDELL

SEQ ID NO: 72 - protein, 466 aa, synthetic construct
QNITEEFYQSTCSAVSKGYLSALRTGWYTSVITIELSNIKENKCNGTDAKVKLIKQELDKYKNAVTELQLLMQSTPATNNQARGSGSGRSLGFLLGVGSAIASGVAVSKVLHLEGEVNKIKSALLSTNKAVVSLSNGVSVLTSKVLDLKNYIDKQLLPIVNKQSCSISNIETVIEFQQKNNRHLEITREFSVNAGVTTPVSTYMLTNSELLSLINDMPITNDQKKLMSNNVQIVRQQSYSIMSIIKEEVLAYVVQLPLYGVIDTPCWKLHTSPLCTTNTKEGSNICLTRTDRGWYCDNAGSVSFFPQAETCKVQSNRVFCDTMNSLTLPSEVNLCNVDIFNPKYDCKIMTSKTDVSSSVITSLGAIVSCYGKTKCTASNKNRGIIKTFSNGCDYVSNKGVDTVSVGNTLYYVNKQEGKSLYVKGEPIINFYDPLVFPSDEFDASISQVNEKINQSLAFIRKSDELL

SEQ ID NO: 73 - protein, 466 aa, synthetic construct
QNITEEFYQSTCSAVSKGYLSALRTGWYTSVITIELSNIKENKCNGTDAKVKLIKQELDKYKNAVTELQLLMQSTPATNNQARGSGSGRSLGFLLGVGSAIASGVAVSKVLHLEGEVNKIKSALLSTNKAVVSLSNGVSVLTSKVLDLKNYIDKQLLPIVNKQSCSISNIETVIEFQQKNNRLLEILREFSVNAGVTTPVSTYMLTNSELLSLINDMPITNDQKKLMSNNVQIVRQQSYSIMSIIKEEVLAYVVQLPLYGVIDTPCWKLHTSPLCTTNTKEGSNICLTRTDRGWYCDNAGSVSFFPQAETCKVQSNRVFCDTMNSLTLPSEVNLCNVDIFNPKYDCKIMTSKTDVSSSVITSLGAIVSCYGKTKCTASNKNRGIIKTFSNGCDYVSNKGVDTVSVGNTLYYVNKQEGKSLYVKGEPIINFYDPLVFPSDEFDASISQVNEKINQSLAFIRKSDELL

SEQ ID NO: 74 - protein, 466 aa, synthetic construct
QNITEEFYQSTCSAVSKGYLSALRTGWYTSVITIELSNIKENKCNGTDAKVKLIKQELDKYKNAVTELQLLMQSTPATNNQARGSGSGRSLGFLLGVGSAIASGVAVSKVLHLEGEVNKIKSALLSTNKAVVSLSNGVSVLTSKVLDLKNYIDKQLLPIVNKQSCSISNIETVIEFQQKNNRLLEIIREFSVNAGVTTPVSTYMLTNSELLSLINDMPITNDQKKLMSNNVQIVRQQSYSIMSIIKEEVLAYVVQLPLYGVIDTPCWKLHTSPLCTTNTKEGSNICLTRTDRGWYCDNAGSVSFFPQAETCKVQSNRVFCDTMNSLTLPSEVNLCNVDIFNPKYDCKIMTSKTDVSSSVITSLGAIVSCYGKTKCTASNKNRGIIKTFSNGCDYVSNKGVDTVSVGNTLYYVNKQEGKSLYVKGEPIINFYDPLVFPSDEFDASISQVNEKINQSLAFIRKSDELL

SEQ ID NO: 75 - protein, 466 aa, synthetic construct
QNITEEFYQSTCSAVSKGYLSALRTGWYTSVITIELSNIKENKCNGTDAKVKLIKQELDKYKNAVTELQLLMQSTPATNNQARGSGSGRSLGFLLGVGSAIASGVAVSKVLHLEGEVNKIKSALLSTNKAVVSLSNGVSVLTSKVLDLKNYIDKQLLPIVNKQSCSISNIETVIEFQQKNNRLLEIMREFSVNAGVTTPVSTYMLTNSELLSLINDMPITNDQKKLMSNNVQIVRQQSYSIMSIIKEEVLAYVVQLPLYGVIDTPCWKLHTSPLCTTNTKEGSNICLTRTDRGWYCDNAGSVSFFPQAETCKVQSNRVFCDTMNSLTLPSEVNLCNVDIFNPKYDCKIMTSKTDVSSSVITSLGAIVSCYGKTKCTASNKNRGIIKTFSNGCDYVSNKGVDTVSVGNTLYYVNKQEGKSLYVKGEPIINFYDPLVFPSDEFDASISQVNEKINQSLAFIRKSDELL

SEQ ID NO: 76 - protein, 466 aa, synthetic construct
QNITEEFYQSTCSAVSKGYLSALRTGWYTSVITIELSNIKENKCNGTDAKVKLIKQELDKYKNAVTELQLLMQSTPATNNQARGSGSGRSLGFLLGVGSAIASGVAVSKVLHLEGEVNKIKSALLSTNKAVVSLSNGVSVLTSKVLDLKNYIDKQLLPIVNKQSCSISNIETVIEFQQKNNRLLEIFREFSVNAGVTTPVSTYMLTNSELLSLINDMPITNDQKKLMSNNVQIVRQQSYSIMSIIKEEVLAYVVQLPLYGVIDTPCWKLHTSPLCTTNTKEGSNICLTRTDRGWYCDNAGSVSFFPQAETCKVQSNRVFCDTMNSLTLPSEVNLCNVDIFNPKYDCKIMTSKTDVSSSVITSLGAIVSCYGKTKCTASNKNRGIIKTFSNGCDYVSNKGVDTVSVGNTLYYVNKQEGKSLYVKGEPIINFYDPLVFPSDEFDASISQVNEKINQSLAFIRKSDELL

SEQ ID NO: 77 - protein, 466 aa, synthetic construct
QNITEEFYQSTCSAVSKGYLSALRTGWYTSVITIELSNIKENKCNGTDAKVKLIKQELDKYKNAVTELQLLMQSTPATNNQARGSGSGRSLGFLLGVGSAIASGVAVSKVLHLEGEVNKIKSALLSTNKAVVSLSNGVSVLTSKVLDLKNYIDKQLLPIVNKQSCSISNIETVIEFQQKNNRLLEIYREFSVNAGVTTPVSTYMLTNSELLSLINDMPITNDQKKLMSNNVQIVRQQSYSIMSIIKEEVLAYVVQLPLYGVIDTPCWKLHTSPLCTTNTKEGSNICLTRTDRGWYCDNAGSVSFFPQAETCKVQSNRVFCDTMNSLTLPSEVNLCNVDIFNPKYDCKIMTSKTDVSSSVITSLGAIVSCYGKTKCTASNKNRGIIKTFSNGCDYVSNKGVDTVSVGNTLYYVNKQEGKSLYVKGEPIINFYDPLVFPSDEFDASISQVNEKINQSLAFIRKSDELL

SEQ ID NO: 78 - protein, 466 aa, synthetic construct
QNITEEFYQSTCSAVSKGYLSALRTGWYTSVITIELSNIKENKCNGTDAKVKLIKQELDKYKNAVTELQLLMQSTPATNNQARGSGSGRSLGFLLGVGSAIASGVAVSKVLHLEGEVNKIKSALLSTNKAVVSLSNGVSVLTSKVLDLKNYIDKQLLPIVNKQSCSISNIETVIEFQQKNNRLLEIWREFSVNAGVTTPVSTYMLTNSELLSLINDMPITNDQKKLMSNNVQIVRQQSYSIMSIIKEEVLAYVVQLPLYGVIDTPCWKLHTSPLCTTNTKEGSNICLTRTDRGWYCDNAGSVSFFPQAETCKVQSNRVFCDTMNSLTLPSEVNLCNVDIFNPKYDCKIMTSKTDVSSSVITSLGAIVSCYGKTKCTASNKNRGIIKTFSNGCDYVSNKGVDTVSVGNTLYYVNKQEGKSLYVKGEPIINFYDPLVFPSDEFDASISQVNEKINQSLAFIRKSDELL

SEQ ID NO: 79 - protein, 466 aa, synthetic construct
QNITEEFYQSTCSAVSKGYLSALRTGWYTSVITIELSNIKENKCNGTDAKVKLIKQELDKYKNAVTELQLLMQSTPATNNQARGSGSGRSLGFLLGVGSAIASGVAVSKVLHLEGEVNKIKSALLSTNKAVVSLSNGVSVLTSKVLDLKNYIDKQLLPIVNKQSCSISNIETVIEFQQKNNRLLEITREFLVNAGVTTPVSTYMLTNSELLSLINDMPITNDQKKLMSNNVQIVRQQSYSIMSIIKEEVLAYVVQLPLYGVIDTPCWKLHTSPLCTTNTKEGSNICLTRTDRGWYCDNAGSVSFFPQAETCKVQSNRVFCDTMNSLTLPSEVNLCNVDIFNPKYDCKIMTSKTDVSSSVITSLGAIVSCYGKTKCTASNKNRGIIKTFSNGCDYVSNKGVDTVSVGNTLYYVNKQEGKSLYVKGEPIINFYDPLVFPSDEFDASISQVNEKINQSLAFIRKSDELL

SEQ ID NO: 80 - protein, 466 aa, synthetic construct
QNITEEFYQSTCSAVSKGYLSALRTGWYTSVITIELSNIKENKCNGTDAKVKLIKQELDKYKNAVTELQLLMQSTPATNNQARGSGSGRSLGFLLGVGSAIASGVAVSKVLHLEGEVNKIKSALLSTNKAVVSLSNGVSVLTSKVLDLKNYIDKQLLPIVNKQSCSISNIETVIEFQQKNNRLLEITREFIVNAGVTTPVSTYMLTNSELLSLINDMPITNDQKKLMSNNVQIVRQQSYSIMSIIKEEVLAYVVQLPLYGVIDTPCWKLHTSPLCTTNTKEGSNICLTRTDRGWYCDNAGSVSFFPQAETCKVQSNRVFCDTMNSLTLPSEVNLCNVDIFNPKYDCKIMTSKTDVSSSVITSLGAIVSCYGKTKCTASNKNRGIIKTFSNGCDYVSNKGVDTVSVGNTLYYVNKQEGKSLYVKGEPIINFYDPLVFPSDEFDASISQVNEKINQSLAFIRKSDELL

SEQ ID NO: 81 - protein, 466 aa, synthetic construct
QNITEEFYQSTCSAVSKGYLSALRTGWYTSVITIELSNIKENKCNGTDAKVKLIKQELDKYKNAVTELQLLMQSTPATNNQARGSGSGRSLGFLLGVGSAIASGVAVSKVLHLEGEVNKIKSALLSTNKAVVSLSNGVSVLTSKVLDLKNYIDKQLLPIVNKQSCSISNIETVIEFQQKNNRLLEITREFMVNAGVTTPVSTYMLTNSELLSLINDMPITNDQKKLMSNNVQIVRQQSYSIMSIIKEEVLAYVVQLPLYGVIDTPCWKLHTSPLCTTNTKEGSNICLTRTDRGWYCDNAGSVSFFPQAETCKVQSNRVFCDTMNSLTLPSEVNLCNVDIFNPKYDCKIMTSKTDVSSSVITSLGAIVSCYGKTKCTASNKNRGIIKTFSNGCDYVSNKGVDTVSVGNTLYYVNKQEGKSLYVKGEPIINFYDPLVFPSDEFDASISQVNEKINQSLAFIRKSDELL

SEQ ID NO: 82 - protein, 466 aa, synthetic construct
QNITEEFYQSTCSAVSKGYLSALRTGWYTSVITIELSNIKENKCNGTDAKVKLIKQELDKYKNAVTELQLLMQSTPATNNQARGSGSGRSLGFLLGVGSAIASGVAVSKVLHLEGEVNKIKSALLSTNKAVVSLSNGVSVLTSKVLDLKNYIDKQLLPIVNKQSCSISNIETVIEFQQKNNRLLEITREFFVNAGVTTPVSTYMLTNSELLSLINDMPITNDQKKLMSNNVQIVRQQSYSIMSIIKEEVLAYVVQLPLYGVIDTPCWKLHTSPLCTTNTKEGSNICLTRTDRGWYCDNAGSVSFFPQAETCKVQSNRVFCDTMNSLTLPSEVNLCNVDIFNPKYDCKIMTSKTDVSSSVITSLGAIVSCYGKTKCTASNKNRGIIKTFSNGCDYVSNKGVDTVSVGNTLYYVNKQEGKSLYVKGEPIINFYDPLVFPSDEFDASISQVNEKINQSLAFIRKSDELL

SEQ ID NO: 83 - protein, 466 aa, synthetic construct
QNITEEFYQSTCSAVSKGYLSALRTGWYTSVITIELSNIKENKCNGTDAKVKLIKQELDKYKNAVTELQLLMQSTPATNNQARGSGSGRSLGFLLGVGSAIASGVAVSKVLHLEGEVNKIKSALLSTNKAVVSLSNGVSVLTSKVLDLKNYIDKQLLPIVNKQSCSISNIETVIEFQQKNNRLLEITREFYVNAGVTTPVSTYMLTNSELLSLINDMPITNDQKKLMSNNVQIVRQQSYSIMSIIKEEVLAYVVQLPLYGVIDTPCWKLHTSPLCTTNTKEGSNICLTRTDRGWYCDNAGSVSFFPQAETCKVQSNRVFCDTMNSLTLPSEVNLCNVDIFNPKYDCKIMTSKTDVSSSVITSLGAIVSCYGKTKCTASNKNRGIIKTFSNGCDYVSNKGVDTVSVGNTLYYVNKQEGKSLYVKGEPIINFYDPLVFPSDEFDASISQVNEKINQSLAFIRKSDELL

SEQ ID NO: 84 - protein, 466 aa, synthetic construct
QNITEEFYQSTCSAVSKGYLSALRTGWYTSVITIELSNIKENKCNGTDAKVKLIKQELDKYKNAVTELQLLMQSTPATNNQARGSGSGRSLGFLLGVGSAIASGVAVSKVLHLEGEVNKIKSALLSTNKAVVSLSNGVSVLTSKVLDLKNYIDKQLLPIVNKQSCSISNIETVIEFQQKNNRLLEITREFWVNAGVTTPVSTYMLTNSELLSLINDMPITNDQKKLMSNNVQIVRQQSYSIMSIIKEEVLAYVVQLPLYGVIDTPCWKLHTSPLCTTNTKEGSNICLTRTDRGWYCDNAGSVSFFPQAETCKVQSNRVFCDTMNSLTLPSEVNLCNVDIFNPKYDCKIMTSKTDVSSSVITSLGAIVSCYGKTKCTASNKNRGIIKTFSNGCDYVSNKGVDTVSVGNTLYYVNKQEGKSLYVKGEPIINFYDPLVFPSDEFDASISQVNEKINQSLAFIRKSDELL

SEQ ID NO: 85 - protein, 466 aa, synthetic construct
QNITEEFYQSTCSAVSKGYLSALRTGWYTSVITIELSNIKENKCNGTDAKVKLIKQLLDKYKNAVTELQLLMQSTPATNNQARGSGSGRSLGFLLGVGSAIASGVAVSKVLHLEGEVNKIKSALLSTNKAVVSLSNGVSVLTSKVLDLKNYIDKQLLPIVNKQSCSISNIETVIEFQQKNNRLLEITREFSVNAGVTTPVSTYMLTNSELLSLINDMPITNDQKKLMSNNVQIVRQQSYSIMSIIKEEVLAYVVQLPLYGVIDTPCWKLHTSPLCTTNTKEGSNICLTRTDRGWYCDNAGSVSFFPQAETCKVQSNRVFCDTMNSLTLPSEVNLCNVDIFNPKYDCKIMTSKTDVSSSVITSLGAIVSCYGKTKCTASNKNRGIIKTFSNGCDYVSNKGVDTVSVGNTLYYVNKQEGKSLYVKGEPIINFYDPLVFPSDEFDASISQVNEKINQSLAFIRKSDELL

SEQ ID NO: 86 - protein, 466 aa, synthetic construct
QNITEEFYQSTCSAVSKGYLSALRTGWYTSVITIELSNIKENKCNGTDAKVKLIKQILDKYKNAVTELQLLMQSTPATNNQARGSGSGRSLGFLLGVGSAIASGVAVSKVLHLEGEVNKIKSALLSTNKAVVSLSNGVSVLTSKVLDLKNYIDKQLLPIVNKQSCSISNIETVIEFQQKNNRLLEITREFSVNAGVTTPVSTYMLTNSELLSLINDMPITNDQKKLMSNNVQIVRQQSYSIMSIIKEEVLAYVVQLPLYGVIDTPCWKLHTSPLCTTNTKEGSNICLTRTDRGWYCDNAGSVSFFPQAETCKVQSNRVFCDTMNSLTLPSEVNLCNVDIFNPKYDCKIMTSKTDVSSSVITSLGAIVSCYGKTKCTASNKNRGIIKTFSNGCDYVSNKGVDTVSVGNTLYYVNKQEGKSLYVKGEPIINFYDPLVFPSDEFDASISQVNEKINQSLAFIRKSDELL

SEQ ID NO: 87 - protein, 466 aa, synthetic construct
QNITEEFYQSTCSAVSKGYLSALRTGWYTSVITIELSNIKENKCNGTDAKVKLIKQMLDKYKNAVTELQLLMQSTPATNNQARGSGSGRSLGFLLGVGSAIASGVAVSKVLHLEGEVNKIKSALLSTNKAVVSLSNGVSVLTSKVLDLKNYIDKQLLPIVNKQSCSISNIETVIEFQQKNNRLLEITREFSVNAGVTTPVSTYMLTNSELLSLINDMPITNDQKKLMSNNVQIVRQQSYSIMSIIKEEVLAYVVQLPLYGVIDTPCWKLHTSPLCTTNTKEGSNICLTRTDRGWYCDNAGSVSFFPQAETCKVQSNRVFCDTMNSLTLPSEVNLCNVDIFNPKYDCKIMTSKTDVSSSVITSLGAIVSCYGKTKCTASNKNRGIIKTFSNGCDYVSNKGVDTVSVGNTLYYVNKQEGKSLYVKGEPIINFYDPLVFPSDEFDASISQVNEKINQSLAFIRKSDELL

SEQ ID NO: 88 - protein, 466 aa, synthetic construct
QNITEEFYQSTCSAVSKGYLSALRTGWYTSVITIELSNIKENKCNGTDAKVKLIKQFLDKYKNAVTELQLLMQSTPATNNQARGSGSGRSLGFLLGVGSAIASGVAVSKVLHLEGEVNKIKSALLSTNKAVVSLSNGVSVLTSKVLDLKNYIDKQLLPIVNKQSCSISNIETVIEFQQKNNRLLEITREFSVNAGVTTPVSTYMLTNSELLSLINDMPITNDQKKLMSNNVQIVRQQSYSIMSIIKEEVLAYVVQLPLYGVIDTPCWKLHTSPLCTTNTKEGSNICLTRTDRGWYCDNAGSVSFFPQAETCKVQSNRVFCDTMNSLTLPSEVNLCNVDIFNPKYDCKIMTSKTDVSSSVITSLGAIVSCYGKTKCTASNKNRGIIKTFSNGCDYVSNKGVDTVSVGNTLYYVNKQEGKSLYVKGEPIINFYDPLVFPSDEFDASISQVNEKINQSLAFIRKSDELL

SEQ ID NO: 89 - protein, 466 aa, synthetic construct
QNITEEFYQSTCSAVSKGYLSALRTGWYTSVITIELSNIKENKCNGTDAKVKLIKQYLDKYKNAVTELQLLMQSTPATNNQARGSGSGRSLGFLLGVGSAIASGVAVSKVLHLEGEVNKIKSALLSTNKAVVSLSNGVSVLTSKVLDLKNYIDKQLLPIVNKQSCSISNIETVIEFQQKNNRLLEITREFSVNAGVTTPVSTYMLTNSELLSLINDMPITNDQKKLMSNNVQIVRQQSYSIMSIIKEEVLAYVVQLPLYGVIDTPCWKLHTSPLCTTNTKEGSNICLTRTDRGWYCDNAGSVSFFPQAETCKVQSNRVFCDTMNSLTLPSEVNLCNVDIFNPKYDCKIMTSKTDVSSSVITSLGAIVSCYGKTKCTASNKNRGIIKTFSNGCDYVSNKGVDTVSVGNTLYYVNKQEGKSLYVKGEPIINFYDPLVFPSDEFDASISQVNEKINQSLAFIRKSDELL

SEQ ID NO: 90 - protein, 466 aa, synthetic construct
QNITEEFYQSTCSAVSKGYLSALRTGWYTSVITIELSNIKENKCNGTDAKVKLIKQWLDKYKNAVTELQLLMQSTPATNNQARGSGSGRSLGFLLGVGSAIASGVAVSKVLHLEGEVNKIKSALLSTNKAVVSLSNGVSVLTSKVLDLKNYIDKQLLPIVNKQSCSISNIETVIEFQQKNNRLLEITREFSVNAGVTTPVSTYMLTNSELLSLINDMPITNDQKKLMSNNVQIVRQQSYSIMSIIKEEVLAYVVQLPLYGVIDTPCWKLHTSPLCTTNTKEGSNICLTRTDRGWYCDNAGSVSFFPQAETCKVQSNRVFCDTMNSLTLPSEVNLCNVDIFNPKYDCKIMTSKTDVSSSVITSLGAIVSCYGKTKCTASNKNRGIIKTFSNGCDYVSNKGVDTVSVGNTLYYVNKQEGKSLYVKGEPIINFYDPLVFPSDEFDASISQVNEKINQSLAFIRKSDELL

SEQ ID NO: 91 - protein, 466 aa, synthetic construct
QNITEEFYQSTCSAVSKGYLSALRTGWYTSVITIELSNIKENKCNGTDAKVKLIKQELDKWKNAVTELQLLMQSTPATNNQARGSGSGRSLGFLLGVGSAIASGVAVSKVLHLEGEVNKIKSALLSTNKAVVSLSNGVSVLTSKVLDLKNYIDKQLLPIVNKQSCSISNIETVIEFQQKNNRLLEITREFSVNAGVTTPVSTYMLTNSELLSLINDMPITNDQKKLMSNNVQIVRQQSYSIMSIIKEEVLAYVVQLPLYGVIDTPCWKLHTSPLCTTNTKEGSNICLTRTDRGWYCDNAGSVSFFPQAETCKVQSNRVFCDTMNSLTLPSEVNLCNVDIFNPKYDCKIMTSKTDVSSSVITSLGAIVSCYGKTKCTASNKNRGIIKTFSNGCDYVSNKGVDTVSVGNTLYYVNKQEGKSLYVKGEPIINFYDPLVFPSDEFDASISQVNEKINQSLAFIRKSDELL

SEQ ID NO: 92 - protein, 466 aa, synthetic construct
QNITEEFYQSTCSAVSKGYLSALRTGWYTSVITIELSNIKENKCNGTDAKVKLIKQELDKYKNLVTELQLLMQSTPATNNQARGSGSGRSLGFLLGVGSAIASGVAVSKVLHLEGEVNKIKSALLSTNKAVVSLSNGVSVLTSKVLDLKNYIDKQLLPIVNKQSCSISNIETVIEFQQKNNRLLEITREFSVNAGVTTPVSTYMLTNSELLSLINDMPITNDQKKLMSNNVQIVRQQSYSIMSIIKEEVLAYVVQLPLYGVIDTPCWKLHTSPLCTTNTKEGSNICLTRTDRGWYCDNAGSVSFFPQAETCKVQSNRVFCDTMNSLTLPSEVNLCNVDIFNPKYDCKIMTSKTDVSSSVITSLGAIVSCYGKTKCTASNKNRGIIKTFSNGCDYVSNKGVDTVSVGNTLYYVNKQEGKSLYVKGEPIINFYDPLVFPSDEFDASISQVNEKINQSLAFIRKSDELL

SEQ ID NO: 93 - protein, 466 aa, synthetic construct
QNITEEFYQSTCSAVSKGYLSALRTGWYTSVITIELSNIKENKCNGTDAKVKLIKQELDKYKNIVTELQLLMQSTPATNNQARGSGSGRSLGFLLGVGSAIASGVAVSKVLHLEGEVNKIKSALLSTNKAVVSLSNGVSVLTSKVLDLKNYIDKQLLPIVNKQSCSISNIETVIEFQQKNNRLLEITREFSVNAGVTTPVSTYMLTNSELLSLINDMPITNDQKKLMSNNVQIVRQQSYSIMSIIKEEVLAYVVQLPLYGVIDTPCWKLHTSPLCTTNTKEGSNICLTRTDRGWYCDNAGSVSFFPQAETCKVQSNRVFCDTMNSLTLPSEVNLCNVDIFNPKYDCKIMTSKTDVSSSVITSLGAIVSCYGKTKCTASNKNRGIIKTFSNGCDYVSNKGVDTVSVGNTLYYVNKQEGKSLYVKGEPIINFYDPLVFPSDEFDASISQVNEKINQSLAFIRKSDELL

SEQ ID NO: 94 - protein, 466 aa, synthetic construct
QNITEEFYQSTCSAVSKGYLSALRTGWYTSVITIELSNIKENKCNGTDAKVKLIKQELDKYKNMVTELQLLMQSTPATNNQARGSGSGRSLGFLLGVGSAIASGVAVSKVLHLEGEVNKIKSALLSTNKAVVSLSNGVSVLTSKVLDLKNYIDKQLLPIVNKQSCSISNIETVIEFQQKNNRLLEITREFSVNAGVTTPVSTYMLTNSELLSLINDMPITNDQKKLMSNNVQIVRQQSYSIMSIIKEEVLAYVVQLPLYGVIDTPCWKLHTSPLCTTNTKEGSNICLTRTDRGWYCDNAGSVSFFPQAETCKVQSNRVFCDTMNSLTLPSEVNLCNVDIFNPKYDCKIMTSKTDVSSSVITSLGAIVSCYGKTKCTASNKNRGIIKTFSNGCDYVSNKGVDTVSVGNTLYYVNKQEGKSLYVKGEPIINFYDPLVFPSDEFDASISQVNEKINQSLAFIRKSDELL

SEQ ID NO: 95 - protein, 466 aa, synthetic construct
QNITEEFYQSTCSAVSKGYLSALRTGWYTSVITIELSNIKENKCNGTDAKVKLIKQELDKYKNFVTELQLLMQSTPATNNQARGSGSGRSLGFLLGVGSAIASGVAVSKVLHLEGEVNKIKSALLSTNKAVVSLSNGVSVLTSKVLDLKNYIDKQLLPIVNKQSCSISNIETVIEFQQKNNRLLEITREFSVNAGVTTPVSTYMLTNSELLSLINDMPITNDQKKLMSNNVQIVRQQSYSIMSIIKEEVLAYVVQLPLYGVIDTPCWKLHTSPLCTTNTKEGSNICLTRTDRGWYCDNAGSVSFFPQAETCKVQSNRVFCDTMNSLTLPSEVNLCNVDIFNPKYDCKIMTSKTDVSSSVITSLGAIVSCYGKTKCTASNKNRGIIKTFSNGCDYVSNKGVDTVSVGNTLYYVNKQEGKSLYVKGEPIINFYDPLVFPSDEFDASISQVNEKINQSLAFIRKSDELL

SEQ ID NO: 96 - protein, 466 aa, synthetic construct
QNITEEFYQSTCSAVSKGYLSALRTGWYTSVITIELSNIKENKCNGTDAKVKLIKQELDKYKNYVTELQLLMQSTPATNNQARGSGSGRSLGFLLGVGSAIASGVAVSKVLHLEGEVNKIKSALLSTNKAVVSLSNGVSVLTSKVLDLKNYIDKQLLPIVNKQSCSISNIETVIEFQQKNNRLLEITREFSVNAGVTTPVSTYMLTNSELLSLINDMPITNDQKKLMSNNVQIVRQQSYSIMSIIKEEVLAYVVQLPLYGVIDTPCWKLHTSPLCTTNTKEGSNICLTRTDRGWYCDNAGSVSFFPQAETCKVQSNRVFCDTMNSLTLPSEVNLCNVDIFNPKYDCKIMTSKTDVSSSVITSLGAIVSCYGKTKCTASNKNRGIIKTFSNGCDYVSNKGVDTVSVGNTLYYVNKQEGKSLYVKGEPIINFYDPLVFPSDEFDASISQVNEKINQSLAFIRKSDELL

SEQ ID NO: 97 - protein, 466 aa, synthetic construct
QNITEEFYQSTCSAVSKGYLSALRTGWYTSVITIELSNIKENKCNGTDAKVKLIKQELDKYKNWVTELQLLMQSTPATNNQARGSGSGRSLGFLLGVGSAIASGVAVSKVLHLEGEVNKIKSALLSTNKAVVSLSNGVSVLTSKVLDLKNYIDKQLLPIVNKQSCSISNIETVIEFQQKNNRLLEITREFSVNAGVTTPVSTYMLTNSELLSLINDMPITNDQKKLMSNNVQIVRQQSYSIMSIIKEEVLAYVVQLPLYGVIDTPCWKLHTSPLCTTNTKEGSNICLTRTDRGWYCDNAGSVSFFPQAETCKVQSNRVFCDTMNSLTLPSEVNLCNVDIFNPKYDCKIMTSKTDVSSSVITSLGAIVSCYGKTKCTASNKNRGIIKTFSNGCDYVSNKGVDTVSVGNTLYYVNKQEGKSLYVKGEPIINFYDPLVFPSDEFDASISQVNEKINQSLAFIRKSDELL

SEQ ID NO: 98 - protein, 466 aa, synthetic construct
QNITEEFYQSTCSAVSKGYLSALRTGWYTSVITIELSNIKENKCNGTDAKVKLIKQELDKYKNAVTLLQLLMQSTPATNNQARGSGSGRSLGFLLGVGSAIASGVAVSKVLHLEGEVNKIKSALLSTNKAVVSLSNGVSVLTSKVLDLKNYIDKQLLPIVNKQSCSISNIETVIEFQQKNNRLLEITREFSVNAGVTTPVSTYMLTNSELLSLINDMPITNDQKKLMSNNVQIVRQQSYSIMSIIKEEVLAYVVQLPLYGVIDTPCWKLHTSPLCTTNTKEGSNICLTRTDRGWYCDNAGSVSFFPQAETCKVQSNRVFCDTMNSLTLPSEVNLCNVDIFNPKYDCKIMTSKTDVSSSVITSLGAIVSCYGKTKCTASNKNRGIIKTFSNGCDYVSNKGVDTVSVGNTLYYVNKQEGKSLYVKGEPIINFYDPLVFPSDEFDASISQVNEKINQSLAFIRKSDELL

SEQ ID NO: 99 - protein, 466 aa, synthetic construct
QNITEEFYQSTCSAVSKGYLSALRTGWYTSVITIELSNIKENKCNGTDAKVKLIKQELDKYKNAVTILQLLMQSTPATNNQARGSGSGRSLGFLLGVGSAIASGVAVSKVLHLEGEVNKIKSALLSTNKAVVSLSNGVSVLTSKVLDLKNYIDKQLLPIVNKQSCSISNIETVIEFQQKNNRLLEITREFSVNAGVTTPVSTYMLTNSELLSLINDMPITNDQKKLMSNNVQIVRQQSYSIMSIIKEEVLAYVVQLPLYGVIDTPCWKLHTSPLCTTNTKEGSNICLTRTDRGWYCDNAGSVSFFPQAETCKVQSNRVFCDTMNSLTLPSEVNLCNVDIFNPKYDCKIMTSKTDVSSSVITSLGAIVSCYGKTKCTASNKNRGIIKTFSNGCDYVSNKGVDTVSVGNTLYYVNKQEGKSLYVKGEPIINFYDPLVFPSDEFDASISQVNEKINQSLAFIRKSDELL

SEQ ID NO: 100 - protein, 466 aa, synthetic construct
QNITEEFYQSTCSAVSKGYLSALRTGWYTSVITIELSNIKENKCNGTDAKVKLIKQELDKYKNAVTMLQLLMQSTPATNNQARGSGSGRSLGFLLGVGSAIASGVAVSKVLHLEGEVNKIKSALLSTNKAVVSLSNGVSVLTSKVLDLKNYIDKQLLPIVNKQSCSISNIETVIEFQQKNNRLLEITREFSVNAGVTTPVSTYMLTNSELLSLINDMPITNDQKKLMSNNVQIVRQQSYSIMSIIKEEVLAYVVQLPLYGVIDTPCWKLHTSPLCTTNTKEGSNICLTRTDRGWYCDNAGSVSFFPQAETCKVQSNRVFCDTMNSLTLPSEVNLCNVDIFNPKYDCKIMTSKTDVSSSVITSLGAIVSCYGKTKCTASNKNRGIIKTFSNGCDYVSNKGVDTVSVGNTLYYVNKQEGKSLYVKGEPIINFYDPLVFPSDEFDASISQVNEKINQSLAFIRKSDELL

SEQ ID NO: 101 - protein, 466 aa, synthetic construct
QNITEEFYQSTCSAVSKGYLSALRTGWYTSVITIELSNIKENKCNGTDAKVKLIKQELDKYKNAVTFLQLLMQSTPATNNQARGSGSGRSLGFLLGVGSAIASGVAVSKVLHLEGEVNKIKSALLSTNKAVVSLSNGVSVLTSKVLDLKNYIDKQLLPIVNKQSCSISNIETVIEFQQKNNRLLEITREFSVNAGVTTPVSTYMLTNSELLSLINDMPITNDQKKLMSNNVQIVRQQSYSIMSIIKEEVLAYVVQLPLYGVIDTPCWKLHTSPLCTTNTKEGSNICLTRTDRGWYCDNAGSVSFFPQAETCKVQSNRVFCDTMNSLTLPSEVNLCNVDIFNPKYDCKIMTSKTDVSSSVITSLGAIVSCYGKTKCTASNKNRGIIKTFSNGCDYVSNKGVDTVSVGNTLYYVNKQEGKSLYVKGEPIINFYDPLVFPSDEFDASISQVNEKINQSLAFIRKSDELL

SEQ ID NO: 102 - protein, 466 aa, synthetic construct
QNITEEFYQSTCSAVSKGYLSALRTGWYTSVITIELSNIKENKCNGTDAKVKLIKQELDKYKNAVTYLQLLMQSTPATNNQARGSGSGRSLGFLLGVGSAIASGVAVSKVLHLEGEVNKIKSALLSTNKAVVSLSNGVSVLTSKVLDLKNYIDKQLLPIVNKQSCSISNIETVIEFQQKNNRLLEITREFSVNAGVTTPVSTYMLTNSELLSLINDMPITNDQKKLMSNNVQIVRQQSYSIMSIIKEEVLAYVVQLPLYGVIDTPCWKLHTSPLCTTNTKEGSNICLTRTDRGWYCDNAGSVSFFPQAETCKVQSNRVFCDTMNSLTLPSEVNLCNVDIFNPKYDCKIMTSKTDVSSSVITSLGAIVSCYGKTKCTASNKNRGIIKTFSNGCDYVSNKGVDTVSVGNTLYYVNKQEGKSLYVKGEPIINFYDPLVFPSDEFDASISQVNEKINQSLAFIRKSDELL

SEQ ID NO: 103 - protein, 466 aa, synthetic construct
QNITEEFYQSTCSAVSKGYLSALRTGWYTSVITIELSNIKENKCNGTDAKVKLIKQELDKYKNAVTWLQLLMQSTPATNNQARGSGSGRSLGFLLGVGSAIASGVAVSKVLHLEGEVNKIKSALLSTNKAVVSLSNGVSVLTSKVLDLKNYIDKQLLPIVNKQSCSISNIETVIEFQQKNNRLLEITREFSVNAGVTTPVSTYMLTNSELLSLINDMPITNDQKKLMSNNVQIVRQQSYSIMSIIKEEVLAYVVQLPLYGVIDTPCWKLHTSPLCTTNTKEGSNICLTRTDRGWYCDNAGSVSFFPQAETCKVQSNRVFCDTMNSLTLPSEVNLCNVDIFNPKYDCKIMTSKTDVSSSVITSLGAIVSCYGKTKCTASNKNRGIIKTFSNGCDYVSNKGVDTVSVGNTLYYVNKQEGKSLYVKGEPIINFYDPLVFPSDEFDASISQVNEKINQSLAFIRKSDELL

SEQ ID NO: 104 - protein, 466 aa, synthetic construct
QNITEEFYQSTCSAVSKGYLSALRTGWYTSVITIELSNIKENKCNGTDAKVKLIKQELDKYKNAVTEMQLLMQSTPATNNQARGSGSGRSLGFLLGVGSAIASGVAVSKVLHLEGEVNKIKSALLSTNKAVVSLSNGVSVLTSKVLDLKNYIDKQLLPIVNKQSCSISNIETVIEFQQKNNRLLEITREFSVNAGVTTPVSTYMLTNSELLSLINDMPITNDQKKLMSNNVQIVRQQSYSIMSIIKEEVLAYVVQLPLYGVIDTPCWKLHTSPLCTTNTKEGSNICLTRTDRGWYCDNAGSVSFFPQAETCKVQSNRVFCDTMNSLTLPSEVNLCNVDIFNPKYDCKIMTSKTDVSSSVITSLGAIVSCYGKTKCTASNKNRGIIKTFSNGCDYVSNKGVDTVSVGNTLYYVNKQEGKSLYVKGEPIINFYDPLVFPSDEFDASISQVNEKINQSLAFIRKSDELL

SEQ ID NO: 105 - protein, 466 aa, synthetic construct
QNITEEFYQSTCSAVSKGYLSALRTGWYTSVITIELSNIKENKCNGTDAKVKLIKQELDKYKNAVTEFQLLMQSTPATNNQARGSGSGRSLGFLLGVGSAIASGVAVSKVLHLEGEVNKIKSALLSTNKAVVSLSNGVSVLTSKVLDLKNYIDKQLLPIVNKQSCSISNIETVIEFQQKNNRLLEITREFSVNAGVTTPVSTYMLTNSELLSLINDMPITNDQKKLMSNNVQIVRQQSYSIMSIIKEEVLAYVVQLPLYGVIDTPCWKLHTSPLCTTNTKEGSNICLTRTDRGWYCDNAGSVSFFPQAETCKVQSNRVFCDTMNSLTLPSEVNLCNVDIFNPKYDCKIMTSKTDVSSSVITSLGAIVSCYGKTKCTASNKNRGIIKTFSNGCDYVSNKGVDTVSVGNTLYYVNKQEGKSLYVKGEPIINFYDPLVFPSDEFDASISQVNEKINQSLAFIRKSDELL

SEQ ID NO: 106 - protein, 466 aa, synthetic construct
QNITEEFYQSTCSAVSKGYLSALRTGWYTSVITIELSNIKENKCNGTDAKVKLIKQELDKYKNAVTEYQLLMQSTPATNNQARGSGSGRSLGFLLGVGSAIASGVAVSKVLHLEGEVNKIKSALLSTNKAVVSLSNGVSVLTSKVLDLKNYIDKQLLPIVNKQSCSISNIETVIEFQQKNNRLLEITREFSVNAGVTTPVSTYMLTNSELLSLINDMPITNDQKKLMSNNVQIVRQQSYSIMSIIKEEVLAYVVQLPLYGVIDTPCWKLHTSPLCTTNTKEGSNICLTRTDRGWYCDNAGSVSFFPQAETCKVQSNRVFCDTMNSLTLPSEVNLCNVDIFNPKYDCKIMTSKTDVSSSVITSLGAIVSCYGKTKCTASNKNRGIIKTFSNGCDYVSNKGVDTVSVGNTLYYVNKQEGKSLYVKGEPIINFYDPLVFPSDEFDASISQVNEKINQSLAFIRKSDELL

SEQ ID NO: 107 - protein, 466 aa, synthetic construct
QNITEEFYQSTCSAVSKGYLSALRTGWYTSVITIELSNIKENKCNGTDAKVKLIKQELDKYKNAVTEWQLLMQSTPATNNQARGSGSGRSLGFLLGVGSAIASGVAVSKVLHLEGEVNKIKSALLSTNKAVVSLSNGVSVLTSKVLDLKNYIDKQLLPIVNKQSCSISNIETVIEFQQKNNRLLEITREFSVNAGVTTPVSTYMLTNSELLSLINDMPITNDQKKLMSNNVQIVRQQSYSIMSIIKEEVLAYVVQLPLYGVIDTPCWKLHTSPLCTTNTKEGSNICLTRTDRGWYCDNAGSVSFFPQAETCKVQSNRVFCDTMNSLTLPSEVNLCNVDIFNPKYDCKIMTSKTDVSSSVITSLGAIVSCYGKTKCTASNKNRGIIKTFSNGCDYVSNKGVDTVSVGNTLYYVNKQEGKSLYVKGEPIINFYDPLVFPSDEFDASISQVNEKINQSLAFIRKSDELL

SEQ ID NO: 108 - protein, 466 aa, synthetic construct
QNITEEFYQSTCSAVSKGYLSALRTGWYTSVITIELSNIKENKCNGTDAKVKLIKQELDKYKNAVTELQLMMQSTPATNNQARGSGSGRSLGFLLGVGSAIASGVAVSKVLHLEGEVNKIKSALLSTNKAVVSLSNGVSVLTSKVLDLKNYIDKQLLPIVNKQSCSISNIETVIEFQQKNNRLLEITREFSVNAGVTTPVSTYMLTNSELLSLINDMPITNDQKKLMSNNVQIVRQQSYSIMSIIKEEVLAYVVQLPLYGVIDTPCWKLHTSPLCTTNTKEGSNICLTRTDRGWYCDNAGSVSFFPQAETCKVQSNRVFCDTMNSLTLPSEVNLCNVDIFNPKYDCKIMTSKTDVSSSVITSLGAIVSCYGKTKCTASNKNRGIIKTFSNGCDYVSNKGVDTVSVGNTLYYVNKQEGKSLYVKGEPIINFYDPLVFPSDEFDASISQVNEKINQSLAFIRKSDELL

SEQ ID NO: 109 - protein, 466 aa, synthetic construct
QNITEEFYQSTCSAVSKGYLSALRTGWYTSVITIELSNIKENKCNGTDAKVKLIKQELDKYKNAVTELQLFMQSTPATNNQARGSGSGRSLGFLLGVGSAIASGVAVSKVLHLEGEVNKIKSALLSTNKAVVSLSNGVSVLTSKVLDLKNYIDKQLLPIVNKQSCSISNIETVIEFQQKNNRLLEITREFSVNAGVTTPVSTYMLTNSELLSLINDMPITNDQKKLMSNNVQIVRQQSYSIMSIIKEEVLAYVVQLPLYGVIDTPCWKLHTSPLCTTNTKEGSNICLTRTDRGWYCDNAGSVSFFPQAETCKVQSNRVFCDTMNSLTLPSEVNLCNVDIFNPKYDCKIMTSKTDVSSSVITSLGAIVSCYGKTKCTASNKNRGIIKTFSNGCDYVSNKGVDTVSVGNTLYYVNKQEGKSLYVKGEPIINFYDPLVFPSDEFDASISQVNEKINQSLAFIRKSDELL

SEQ ID NO: 110 - protein, 466 aa, synthetic construct
QNITEEFYQSTCSAVSKGYLSALRTGWYTSVITIELSNIKENKCNGTDAKVKLIKQELDKYKNAVTELQLYMQSTPATNNQARGSGSGRSLGFLLGVGSAIASGVAVSKVLHLEGEVNKIKSALLSTNKAVVSLSNGVSVLTSKVLDLKNYIDKQLLPIVNKQSCSISNIETVIEFQQKNNRLLEITREFSVNAGVTTPVSTYMLTNSELLSLINDMPITNDQKKLMSNNVQIVRQQSYSIMSIIKEEVLAYVVQLPLYGVIDTPCWKLHTSPLCTTNTKEGSNICLTRTDRGWYCDNAGSVSFFPQAETCKVQSNRVFCDTMNSLTLPSEVNLCNVDIFNPKYDCKIMTSKTDVSSSVITSLGAIVSCYGKTKCTASNKNRGIIKTFSNGCDYVSNKGVDTVSVGNTLYYVNKQEGKSLYVKGEPIINFYDPLVFPSDEFDASISQVNEKINQSLAFIRKSDELL

SEQ ID NO: 111 - protein, 466 aa, synthetic construct
QNITEEFYQSTCSAVSKGYLSALRTGWYTSVITIELSNIKENKCNGTDAKVKLIKQELDKYKNAVTELQLWMQSTPATNNQARGSGSGRSLGFLLGVGSAIASGVAVSKVLHLEGEVNKIKSALLSTNKAVVSLSNGVSVLTSKVLDLKNYIDKQLLPIVNKQSCSISNIETVIEFQQKNNRLLEITREFSVNAGVTTPVSTYMLTNSELLSLINDMPITNDQKKLMSNNVQIVRQQSYSIMSIIKEEVLAYVVQLPLYGVIDTPCWKLHTSPLCTTNTKEGSNICLTRTDRGWYCDNAGSVSFFPQAETCKVQSNRVFCDTMNSLTLPSEVNLCNVDIFNPKYDCKIMTSKTDVSSSVITSLGAIVSCYGKTKCTASNKNRGIIKTFSNGCDYVSNKGVDTVSVGNTLYYVNKQEGKSLYVKGEPIINFYDPLVFPSDEFDASISQVNEKINQSLAFIRKSDELL

SEQ ID NO: 112 - protein, 466 aa, synthetic construct
QNITEEFYQSTCSAVSKGYLSALRTGWYTSVITIELSNIKENKCNGTDAKVKLIKQELDKYKNAVTELQLLMQSTPATNNQARGSGSGRSLGFLLGVGSAIASGVAVSKVLHLEGEVNKIKSALLSTNKAVVSLSNGVSVLTSKVMDLKNYIDKQLLPIVNKQSCSISNIETVIEFQQKNNRLLEITREFSVNAGVTTPVSTYMLTNSELLSLINDMPITNDQKKLMSNNVQIVRQQSYSIMSIIKEEVLAYVVQLPLYGVIDTPCWKLHTSPLCTTNTKEGSNICLTRTDRGWYCDNAGSVSFFPQAETCKVQSNRVFCDTMNSLTLPSEVNLCNVDIFNPKYDCKIMTSKTDVSSSVITSLGAIVSCYGKTKCTASNKNRGIIKTFSNGCDYVSNKGVDTVSVGNTLYYVNKQEGKSLYVKGEPIINFYDPLVFPSDEFDASISQVNEKINQSLAFIRKSDELL

SEQ ID NO: 113 - protein, 466 aa, synthetic construct
QNITEEFYQSTCSAVSKGYLSALRTGWYTSVITIELSNIKENKCNGTDAKVKLIKQELDKYKNAVTELQLLMQSTPATNNQARGSGSGRSLGFLLGVGSAIASGVAVSKVLHLEGEVNKIKSALLSTNKAVVSLSNGVSVLTSKVFDLKNYIDKQLLPIVNKQSCSISNIETVIEFQQKNNRLLEITREFSVNAGVTTPVSTYMLTNSELLSLINDMPITNDQKKLMSNNVQIVRQQSYSIMSIIKEEVLAYVVQLPLYGVIDTPCWKLHTSPLCTTNTKEGSNICLTRTDRGWYCDNAGSVSFFPQAETCKVQSNRVFCDTMNSLTLPSEVNLCNVDIFNPKYDCKIMTSKTDVSSSVITSLGAIVSCYGKTKCTASNKNRGIIKTFSNGCDYVSNKGVDTVSVGNTLYYVNKQEGKSLYVKGEPIINFYDPLVFPSDEFDASISQVNEKINQSLAFIRKSDELL

SEQ ID NO: 114 - protein, 466 aa, synthetic construct
QNITEEFYQSTCSAVSKGYLSALRTGWYTSVITIELSNIKENKCNGTDAKVKLIKQELDKYKNAVTELQLLMQSTPATNNQARGSGSGRSLGFLLGVGSAIASGVAVSKVLHLEGEVNKIKSALLSTNKAVVSLSNGVSVLTSKVYDLKNYIDKQLLPIVNKQSCSISNIETVIEFQQKNNRLLEITREFSVNAGVTTPVSTYMLTNSELLSLINDMPITNDQKKLMSNNVQIVRQQSYSIMSIIKEEVLAYVVQLPLYGVIDTPCWKLHTSPLCTTNTKEGSNICLTRTDRGWYCDNAGSVSFFPQAETCKVQSNRVFCDTMNSLTLPSEVNLCNVDIFNPKYDCKIMTSKTDVSSSVITSLGAIVSCYGKTKCTASNKNRGIIKTFSNGCDYVSNKGVDTVSVGNTLYYVNKQEGKSLYVKGEPIINFYDPLVFPSDEFDASISQVNEKINQSLAFIRKSDELL

SEQ ID NO: 115 - protein, 466 aa, synthetic construct
QNITEEFYQSTCSAVSKGYLSALRTGWYTSVITIELSNIKENKCNGTDAKVKLIKQELDKYKNAVTELQLLMQSTPATNNQARGSGSGRSLGFLLGVGSAIASGVAVSKVLHLEGEVNKIKSALLSTNKAVVSLSNGVSVLTSKVWDLKNYIDKQLLPIVNKQSCSISNIETVIEFQQKNNRLLEITREFSVNAGVTTPVSTYMLTNSELLSLINDMPITNDQKKLMSNNVQIVRQQSYSIMSIIKEEVLAYVVQLPLYGVIDTPCWKLHTSPLCTTNTKEGSNICLTRTDRGWYCDNAGSVSFFPQAETCKVQSNRVFCDTMNSLTLPSEVNLCNVDIFNPKYDCKIMTSKTDVSSSVITSLGAIVSCYGKTKCTASNKNRGIIKTFSNGCDYVSNKGVDTVSVGNTLYYVNKQEGKSLYVKGEPIINFYDPLVFPSDEFDASISQVNEKINQSLAFIRKSDELL

SEQ ID NO: 116 - protein, 466 aa, synthetic construct
QNITEEFYQSTCSAVSKGYLSALRTGWYTSVITIELSNIKENKCNGTDAKVKLIKQELDKYKNAVTELQLLMQSTPATNNQARGSGSGRSLGFLLGVGSAIASGVAVSKVLHLEGEVNKIKSALLSTNKAVVSLSNGVSVLTSKVLDMKNYIDKQLLPIVNKQSCSISNIETVIEFQQKNNRLLEITREFSVNAGVTTPVSTYMLTNSELLSLINDMPITNDQKKLMSNNVQIVRQQSYSIMSIIKEEVLAYVVQLPLYGVIDTPCWKLHTSPLCTTNTKEGSNICLTRTDRGWYCDNAGSVSFFPQAETCKVQSNRVFCDTMNSLTLPSEVNLCNVDIFNPKYDCKIMTSKTDVSSSVITSLGAIVSCYGKTKCTASNKNRGIIKTFSNGCDYVSNKGVDTVSVGNTLYYVNKQEGKSLYVKGEPIINFYDPLVFPSDEFDASISQVNEKINQSLAFIRKSDELL

SEQ ID NO: 117 - protein, 466 aa, synthetic construct
QNITEEFYQSTCSAVSKGYLSALRTGWYTSVITIELSNIKENKCNGTDAKVKLIKQELDKYKNAVTELQLLMQSTPATNNQARGSGSGRSLGFLLGVGSAIASGVAVSKVLHLEGEVNKIKSALLSTNKAVVSLSNGVSVLTSKVLDFKNYIDKQLLPIVNKQSCSISNIETVIEFQQKNNRLLEITREFSVNAGVTTPVSTYMLTNSELLSLINDMPITNDQKKLMSNNVQIVRQQSYSIMSIIKEEVLAYVVQLPLYGVIDTPCWKLHTSPLCTTNTKEGSNICLTRTDRGWYCDNAGSVSFFPQAETCKVQSNRVFCDTMNSLTLPSEVNLCNVDIFNPKYDCKIMTSKTDVSSSVITSLGAIVSCYGKTKCTASNKNRGIIKTFSNGCDYVSNKGVDTVSVGNTLYYVNKQEGKSLYVKGEPIINFYDPLVFPSDEFDASISQVNEKINQSLAFIRKSDELL

SEQ ID NO: 118 - protein, 466 aa, synthetic construct
QNITEEFYQSTCSAVSKGYLSALRTGWYTSVITIELSNIKENKCNGTDAKVKLIKQELDKYKNAVTELQLLMQSTPATNNQARGSGSGRSLGFLLGVGSAIASGVAVSKVLHLEGEVNKIKSALLSTNKAVVSLSNGVSVLTSKVLDYKNYIDKQLLPIVNKQSCSISNIETVIEFQQKNNRLLEITREFSVNAGVTTPVSTYMLTNSELLSLINDMPITNDQKKLMSNNVQIVRQQSYSIMSIIKEEVLAYVVQLPLYGVIDTPCWKLHTSPLCTTNTKEGSNICLTRTDRGWYCDNAGSVSFFPQAETCKVQSNRVFCDTMNSLTLPSEVNLCNVDIFNPKYDCKIMTSKTDVSSSVITSLGAIVSCYGKTKCTASNKNRGIIKTFSNGCDYVSNKGVDTVSVGNTLYYVNKQEGKSLYVKGEPIINFYDPLVFPSDEFDASISQVNEKINQSLAFIRKSDELL

SEQ ID NO: 119 - protein, 466 aa, synthetic construct
QNITEEFYQSTCSAVSKGYLSALRTGWYTSVITIELSNIKENKCNGTDAKVKLIKQELDKYKNAVTELQLLMQSTPATNNQARGSGSGRSLGFLLGVGSAIASGVAVSKVLHLEGEVNKIKSALLSTNKAVVSLSNGVSVLTSKVLDWKNYIDKQLLPIVNKQSCSISNIETVIEFQQKNNRLLEITREFSVNAGVTTPVSTYMLTNSELLSLINDMPITNDQKKLMSNNVQIVRQQSYSIMSIIKEEVLAYVVQLPLYGVIDTPCWKLHTSPLCTTNTKEGSNICLTRTDRGWYCDNAGSVSFFPQAETCKVQSNRVFCDTMNSLTLPSEVNLCNVDIFNPKYDCKIMTSKTDVSSSVITSLGAIVSCYGKTKCTASNKNRGIIKTFSNGCDYVSNKGVDTVSVGNTLYYVNKQEGKSLYVKGEPIINFYDPLVFPSDEFDASISQVNEKINQSLAFIRKSDELL

SEQ ID NO: 120 - protein, 466 aa, synthetic construct
QNITEEFYQSTCSAVSKGYLSALRTGWYTSVITIELSNIKENKCNGTDAKVKLIKQELDKYKNAVTELQLLMQSTPATNNQARGSGSGRSLGFLLGVGSAIASGVAVSKVLHLEGEVNKIKSALLSTNKAVVSLSNGVSVLTSKVLDLKNYMDKQLLPIVNKQSCSISNIETVIEFQQKNNRLLEITREFSVNAGVTTPVSTYMLTNSELLSLINDMPITNDQKKLMSNNVQIVRQQSYSIMSIIKEEVLAYVVQLPLYGVIDTPCWKLHTSPLCTTNTKEGSNICLTRTDRGWYCDNAGSVSFFPQAETCKVQSNRVFCDTMNSLTLPSEVNLCNVDIFNPKYDCKIMTSKTDVSSSVITSLGAIVSCYGKTKCTASNKNRGIIKTFSNGCDYVSNKGVDTVSVGNTLYYVNKQEGKSLYVKGEPIINFYDPLVFPSDEFDASISQVNEKINQSLAFIRKSDELL

SEQ ID NO: 121 - protein, 466 aa, synthetic construct
QNITEEFYQSTCSAVSKGYLSALRTGWYTSVITIELSNIKENKCNGTDAKVKLIKQELDKYKNAVTELQLLMQSTPATNNQARGSGSGRSLGFLLGVGSAIASGVAVSKVLHLEGEVNKIKSALLSTNKAVVSLSNGVSVLTSKVLDLKNYFDKQLLPIVNKQSCSISNIETVIEFQQKNNRLLEITREFSVNAGVTTPVSTYMLTNSELLSLINDMPITNDQKKLMSNNVQIVRQQSYSIMSIIKEEVLAYVVQLPLYGVIDTPCWKLHTSPLCTTNTKEGSNICLTRTDRGWYCDNAGSVSFFPQAETCKVQSNRVFCDTMNSLTLPSEVNLCNVDIFNPKYDCKIMTSKTDVSSSVITSLGAIVSCYGKTKCTASNKNRGIIKTFSNGCDYVSNKGVDTVSVGNTLYYVNKQEGKSLYVKGEPIINFYDPLVFPSDEFDASISQVNEKINQSLAFIRKSDELL

SEQ ID NO: 122 - protein, 466 aa, synthetic construct
QNITEEFYQSTCSAVSKGYLSALRTGWYTSVITIELSNIKENKCNGTDAKVKLIKQELDKYKNAVTELQLLMQSTPATNNQARGSGSGRSLGFLLGVGSAIASGVAVSKVLHLEGEVNKIKSALLSTNKAVVSLSNGVSVLTSKVLDLKNYYDKQLLPIVNKQSCSISNIETVIEFQQKNNRLLEITREFSVNAGVTTPVSTYMLTNSELLSLINDMPITNDQKKLMSNNVQIVRQQSYSIMSIIKEEVLAYVVQLPLYGVIDTPCWKLHTSPLCTTNTKEGSNICLTRTDRGWYCDNAGSVSFFPQAETCKVQSNRVFCDTMNSLTLPSEVNLCNVDIFNPKYDCKIMTSKTDVSSSVITSLGAIVSCYGKTKCTASNKNRGIIKTFSNGCDYVSNKGVDTVSVGNTLYYVNKQEGKSLYVKGEPIINFYDPLVFPSDEFDASISQVNEKINQSLAFIRKSDELL

SEQ ID NO: 123 - protein, 466 aa, synthetic construct
QNITEEFYQSTCSAVSKGYLSALRTGWYTSVITIELSNIKENKCNGTDAKVKLIKQELDKYKNAVTELQLLMQSTPATNNQARGSGSGRSLGFLLGVGSAIASGVAVSKVLHLEGEVNKIKSALLSTNKAVVSLSNGVSVLTSKVLDLKNYWDKQLLPIVNKQSCSISNIETVIEFQQKNNRLLEITREFSVNAGVTTPVSTYMLTNSELLSLINDMPITNDQKKLMSNNVQIVRQQSYSIMSIIKEEVLAYVVQLPLYGVIDTPCWKLHTSPLCTTNTKEGSNICLTRTDRGWYCDNAGSVSFFPQAETCKVQSNRVFCDTMNSLTLPSEVNLCNVDIFNPKYDCKIMTSKTDVSSSVITSLGAIVSCYGKTKCTASNKNRGIIKTFSNGCDYVSNKGVDTVSVGNTLYYVNKQEGKSLYVKGEPIINFYDPLVFPSDEFDASISQVNEKINQSLAFIRKSDELL

SEQ ID NO: 124 - protein, 466 aa, synthetic construct
QNITEEFYQSTCSAVSKGYLSALRTGWYTSVITIELSNIKENKCNGTDAKVKLIKQELDKYKNAVTELQLLMQSTPATNNQARGSGSGRSLGFLLGVGSAIASGVAVSKVLHLEGEVNKIKSALLSTNKAVVSLSNGVSVLTVKVLDLKNYIDKQLLPIVNKQSCSISNIETVIEFQQKNNRLLEITREFSVNAGVTTPVSTYMLTNSELLSLINDMPITNDQKKLMSNNVQIVRQQSYSIMSIIKEEVLAYVVQLPLYGVIDTPCWKLHTSPLCTTNTKEGSNICLTRTDRGWYCDNAGSVSFFPQAETCKVQSNRVFCDTMNSLTLPSEVNLCNVDIFNPKYDCKIMTSKTDVSSSVITSLGAIVSCYGKTKCTASNKNRGIIKTFSNGCDYVSNKGVDTVSVGNTLYYVNKQEGKSLYVKGEPIINFYDPLVFPSDEFDASISQVNEKINQSLAFIRKSDELL

SEQ ID NO: 125 - protein, 466 aa, synthetic construct
QNITEEFYQSTCSAVSKGYLSALRTGWYTSVITIELSNIKENKCNGTDAKVKLIKQELDKYKNAVTELQLLMQSTPATNNQARGSGSGRSLGFMLGVGSAIASGVAVSKVLHLEGEVNKIKSALLSTNKAVVSLSNGVSVLTSKVLDLKNYIDKQLLPIVNKQSCSISNIETVIEFQQKNNRLLEITREFSVNAGVTTPVSTYMLTNSELLSLINDMPITNDQKKLMSNNVQIVRQQSYSIMSIIKEEVLAYVVQLPLYGVIDTPCWKLHTSPLCTTNTKEGSNICLTRTDRGWYCDNAGSVSFFPQAETCKVQSNRVFCDTMNSLTLPSEVNLCNVDIFNPKYDCKIMTSKTDVSSSVITSLGAIVSCYGKTKCTASNKNRGIIKTFSNGCDYVSNKGVDTVSVGNTLYYVNKQEGKSLYVKGEPIINFYDPLVFPSDEFDASISQVNEKINQSLAFIRKSDELL

SEQ ID NO: 126 - protein, 466 aa, synthetic construct
QNITEEFYQSTCSAVSKGYLSALRTGWYTSVITIELSNIKENKCNGTDAKVKLIKQELDKYKNAVTELQLLMQSTPATNNQARGSGSGRSLGFFLGVGSAIASGVAVSKVLHLEGEVNKIKSALLSTNKAVVSLSNGVSVLTSKVLDLKNYIDKQLLPIVNKQSCSISNIETVIEFQQKNNRLLEITREFSVNAGVTTPVSTYMLTNSELLSLINDMPITNDQKKLMSNNVQIVRQQSYSIMSIIKEEVLAYVVQLPLYGVIDTPCWKLHTSPLCTTNTKEGSNICLTRTDRGWYCDNAGSVSFFPQAETCKVQSNRVFCDTMNSLTLPSEVNLCNVDIFNPKYDCKIMTSKTDVSSSVITSLGAIVSCYGKTKCTASNKNRGIIKTFSNGCDYVSNKGVDTVSVGNTLYYVNKQEGKSLYVKGEPIINFYDPLVFPSDEFDASISQVNEKINQSLAFIRKSDELL

SEQ ID NO: 127 - protein, 466 aa, synthetic construct
QNITEEFYQSTCSAVSKGYLSALRTGWYTSVITIELSNIKENKCNGTDAKVKLIKQELDKYKNAVTELQLLMQSTPATNNQARGSGSGRSLGFYLGVGSAIASGVAVSKVLHLEGEVNKIKSALLSTNKAVVSLSNGVSVLTSKVLDLKNYIDKQLLPIVNKQSCSISNIETVIEFQQKNNRLLEITREFSVNAGVTTPVSTYMLTNSELLSLINDMPITNDQKKLMSNNVQIVRQQSYSIMSIIKEEVLAYVVQLPLYGVIDTPCWKLHTSPLCTTNTKEGSNICLTRTDRGWYCDNAGSVSFFPQAETCKVQSNRVFCDTMNSLTLPSEVNLCNVDIFNPKYDCKIMTSKTDVSSSVITSLGAIVSCYGKTKCTASNKNRGIIKTFSNGCDYVSNKGVDTVSVGNTLYYVNKQEGKSLYVKGEPIINFYDPLVFPSDEFDASISQVNEKINQSLAFIRKSDELL

SEQ ID NO: 128 - protein, 466 aa, synthetic construct
QNITEEFYQSTCSAVSKGYLSALRTGWYTSVITIELSNIKENKCNGTDAKVKLIKQELDKYKNAVTELQLLMQSTPATNNQARGSGSGRSLGFWLGVGSAIASGVAVSKVLHLEGEVNKIKSALLSTNKAVVSLSNGVSVLTSKVLDLKNYIDKQLLPIVNKQSCSISNIETVIEFQQKNNRLLEITREFSVNAGVTTPVSTYMLTNSELLSLINDMPITNDQKKLMSNNVQIVRQQSYSIMSIIKEEVLAYVVQLPLYGVIDTPCWKLHTSPLCTTNTKEGSNICLTRTDRGWYCDNAGSVSFFPQAETCKVQSNRVFCDTMNSLTLPSEVNLCNVDIFNPKYDCKIMTSKTDVSSSVITSLGAIVSCYGKTKCTASNKNRGIIKTFSNGCDYVSNKGVDTVSVGNTLYYVNKQEGKSLYVKGEPIINFYDPLVFPSDEFDASISQVNEKINQSLAFIRKSDELL

SEQ ID NO: 129 - protein, 466 aa, synthetic construct
QNITEEFYQSTCSAVSKGYLSALRTGWYTSVITIELSNIKENKCNGTDAKVKLIKQELDKYKNAVTELQLLMQSTPATNNQARGSGSGRSLGFLLGVGSAIASGVAVSKVLHLEGEVNKIKSALLSTNKAVVSLSNGVSVLTSKVLDLKNYIDKQLLPIVNKQSCSISNIETVIEFQQKNNRLLEITREFSVNAGVTTPVSTYMLTNSELLSLINDMPITNDQKKLMSNNVQIVRQQSYSIMSIIKEEVLAYVVQLPLYGVIDTPCWKLHTSPLCTTNTKEGSNICLTRTDRGWYCDNAGSVSFFPQAETCKVQSNRVFCDTMNSMTLPSEVNLCNVDIFNPKYDCKIMTSKTDVSSSVITSLGAIVSCYGKTKCTASNKNRGIIKTFSNGCDYVSNKGVDTVSVGNTLYYVNKQEGKSLYVKGEPIINFYDPLVFPSDEFDASISQVNEKINQSLAFIRKSDELL

SEQ ID NO: 130 - protein, 466 aa, synthetic construct
QNITEEFYQSTCSAVSKGYLSALRTGWYTSVITIELSNIKENKCNGTDAKVKLIKQELDKYKNAVTELQLLMQSTPATNNQARGSGSGRSLGFLLGVGSAIASGVAVSKVLHLEGEVNKIKSALLSTNKAVVSLSNGVSVLTSKVLDLKNYIDKQLLPIVNKQSCSISNIETVIEFQQKNNRLLEITREFSVNAGVTTPVSTYMLTNSELLSLINDMPITNDQKKLMSNNVQIVRQQSYSIMSIIKEEVLAYVVQLPLYGVIDTPCWKLHTSPLCTTNTKEGSNICLTRTDRGWYCDNAGSVSFFPQAETCKVQSNRVFCDTMNSFTLPSEVNLCNVDIFNPKYDCKIMTSKTDVSSSVITSLGAIVSCYGKTKCTASNKNRGIIKTFSNGCDYVSNKGVDTVSVGNTLYYVNKQEGKSLYVKGEPIINFYDPLVFPSDEFDASISQVNEKINQSLAFIRKSDELL

SEQ ID NO: 131 - protein, 466 aa, synthetic construct
QNITEEFYQSTCSAVSKGYLSALRTGWYTSVITIELSNIKENKCNGTDAKVKLIKQELDKYKNAVTELQLLMQSTPATNNQARGSGSGRSLGFLLGVGSAIASGVAVSKVLHLEGEVNKIKSALLSTNKAVVSLSNGVSVLTSKVLDLKNYIDKQLLPIVNKQSCSISNIETVIEFQQKNNRLLEITREFSVNAGVTTPVSTYMLTNSELLSLINDMPITNDQKKLMSNNVQIVRQQSYSIMSIIKEEVLAYVVQLPLYGVIDTPCWKLHTSPLCTTNTKEGSNICLTRTDRGWYCDNAGSVSFFPQAETCKVQSNRVFCDTMNSYTLPSEVNLCNVDIFNPKYDCKIMTSKTDVSSSVITSLGAIVSCYGKTKCTASNKNRGIIKTFSNGCDYVSNKGVDTVSVGNTLYYVNKQEGKSLYVKGEPIINFYDPLVFPSDEFDASISQVNEKINQSLAFIRKSDELL

SEQ ID NO: 132 - protein, 466 aa, synthetic construct
QNITEEFYQSTCSAVSKGYLSALRTGWYTSVITIELSNIKENKCNGTDAKVKLIKQELDKYKNAVTELQLLMQSTPATNNQARGSGSGRSLGFLLGVGSAIASGVAVSKVLHLEGEVNKIKSALLSTNKAVVSLSNGVSVLTSKVLDLKNYIDKQLLPIVNKQSCSISNIETVIEFQQKNNRLLEITREFSVNAGVTTPVSTYMLTNSELLSLINDMPITNDQKKLMSNNVQIVRQQSYSIMSIIKEEVLAYVVQLPLYGVIDTPCWKLHTSPLCTTNTKEGSNICLTRTDRGWYCDNAGSVSFFPQAETCKVQSNRVFCDTMNSWTLPSEVNLCNVDIFNPKYDCKIMTSKTDVSSSVITSLGAIVSCYGKTKCTASNKNRGIIKTFSNGCDYVSNKGVDTVSVGNTLYYVNKQEGKSLYVKGEPIINFYDPLVFPSDEFDASISQVNEKINQSLAFIRKSDELL

SEQ ID NO: 133 - protein, 466 aa, synthetic construct
QNITEEFYQSTCSAVSKGYLSALRTGWYTSVITIELSNIKENKCNGTDAKVKLIKQELDKYKNAVTELQLLMQSTPATNNQARGSGSGRSLGFLLGVGSAIASGVAVSKVLHLEGEVNKIKSALLSTNKAVVSLSNGVSVLTSKVLDLKNYIDKQLLPIVNKQSCSISNIETVIEFQQKFNRFLEITREFSVNAGVTTPVSTYMLTNSELLSLINDMPITNDQKKLMSNNVQIVRQQSYSIMSIIKEEVLAYVVQLPLYGVIDTPCWKLHTSPLCTTNTKEGSNICLTRTDRGWYCDNAGSVSFFPQAETCKVQSNRVFCDTMNSLTLPSEVNLCNVDIFNPKYDCKIMTSKTDVSSSVITSLGAIVSCYGKTKCTASNKNRGIIKTFSNGCDYVSNKGVDTVSVGNTLYYVNKQEGKSLYVKGEPIINFYDPLVFPSDEFDASISQVNEKINQSLAFIRKSDELL

SEQ ID NO: 134 - protein, 466 aa, synthetic construct
QNITEEFYQSTCSAVSKGYLSALRTGWYTSVITIELSNIKENKCNGTDAKVKLIKQLLDKYKNAVTELQLLMQSTPATNNQARGSGSGRSLGFLLGVGSAIASGVAVSKVLHLEGEVNKIKSALLSTNKAVVSLSNGVSVLTSKVLDLKNYIDKQLLPIVNKQSCSISNIETVIEFQQKMNRLLEITREFSVNAGVTTPVSTYMLTNSELLSLINDMPITNDQKKLMSNNVQIVRQQSYSIMSIIKEEVLAYVVQLPLYGVIDTPCWKLHTSPLCTTNTKEGSNICLTRTDRGWYCDNAGSVSFFPQAETCKVQSNRVFCDTMNSLTLPSEVNLCNVDIFNPKYDCKIMTSKTDVSSSVITSLGAIVSCYGKTKCTASNKNRGIIKTFSNGCDYVSNKGVDTVSVGNTLYYVNKQEGKSLYVKGEPIINFYDPLVFPSDEFDASISQVNEKINQSLAFIRKSDELL

SEQ ID NO: 135 - protein, 466 aa, synthetic construct
QNITEEFYQSTCSAVSKGYLSALRTGWYTSVITIELSNIKENKCNGTDAKVKLIKQELDKYKNLVTELQLLMQSTPATNNQARGSGSGRSLGFLLGVGSAIASGVAVSKVLHLEGEVNKIKSALLSTNKAVVSLSNGVSVLTSKVLDLKNYIDKQLLPIVNKQSCSISNIETVIEFQQKMNRLLEITREFSVNAGVTTPVSTYMLTNSELLSLINDMPITNDQKKLMSNNVQIVRQQSYSIMSIIKEEVLAYVVQLPLYGVIDTPCWKLHTSPLCTTNTKEGSNICLTRTDRGWYCDNAGSVSFFPQAETCKVQSNRVFCDTMNSLTLPSEVNLCNVDIFNPKYDCKIMTSKTDVSSSVITSLGAIVSCYGKTKCTASNKNRGIIKTFSNGCDYVSNKGVDTVSVGNTLYYVNKQEGKSLYVKGEPIINFYDPLVFPSDEFDASISQVNEKINQSLAFIRKSDELL

SEQ ID NO: 136 - protein, 466 aa, synthetic construct
QNITEEFYQSTCSAVSKGYLSALRTGWYTSVITIELSNIKENKCNGTDAKVKLIKQELDKYKNAVTEFQLLMQSTPATNNQARGSGSGRSLGFLLGVGSAIASGVAVSKVLHLEGEVNKIKSALLSTNKAVVSLSNGVSVLTSKVLDLKNYIDKQLLPIVNKQSCSISNIETVIEFQQKMNRLLEITREFSVNAGVTTPVSTYMLTNSELLSLINDMPITNDQKKLMSNNVQIVRQQSYSIMSIIKEEVLAYVVQLPLYGVIDTPCWKLHTSPLCTTNTKEGSNICLTRTDRGWYCDNAGSVSFFPQAETCKVQSNRVFCDTMNSLTLPSEVNLCNVDIFNPKYDCKIMTSKTDVSSSVITSLGAIVSCYGKTKCTASNKNRGIIKTFSNGCDYVSNKGVDTVSVGNTLYYVNKQEGKSLYVKGEPIINFYDPLVFPSDEFDASISQVNEKINQSLAFIRKSDELL

SEQ ID NO: 137 - protein, 466 aa, synthetic construct
QNITEEFYQSTCSAVSKGYLSALRTGWYTSVITIELSNIKENKCNGTDAKVKLIKQELDKYKNAVTELQLMMQSTPATNNQARGSGSGRSLGFLLGVGSAIASGVAVSKVLHLEGEVNKIKSALLSTNKAVVSLSNGVSVLTSKVLDLKNYIDKQLLPIVNKQSCSISNIETVIEFQQKMNRLLEITREFSVNAGVTTPVSTYMLTNSELLSLINDMPITNDQKKLMSNNVQIVRQQSYSIMSIIKEEVLAYVVQLPLYGVIDTPCWKLHTSPLCTTNTKEGSNICLTRTDRGWYCDNAGSVSFFPQAETCKVQSNRVFCDTMNSLTLPSEVNLCNVDIFNPKYDCKIMTSKTDVSSSVITSLGAIVSCYGKTKCTASNKNRGIIKTFSNGCDYVSNKGVDTVSVGNTLYYVNKQEGKSLYVKGEPIINFYDPLVFPSDEFDASISQVNEKINQSLAFIRKSDELL

SEQ ID NO: 138 - protein, 466 aa, synthetic construct
QNITEEFYQSTCSAVSKGYLSALRTGWYTSVITIELSNIKENKCNGTDAKVKLIKQELDKYKNFVTELQLLMQSTPATNNQARGSGSGRSLGFLLGVGSAIASGVAVSKVLHLEGEVNKIKSALLSTNKAVVSLSNGVSVLTSKVLDLKNYIDKQLLPIVNKQSCSISNIETVIEFQQKNNRFLEITREFSVNAGVTTPVSTYMLTNSELLSLINDMPITNDQKKLMSNNVQIVRQQSYSIMSIIKEEVLAYVVQLPLYGVIDTPCWKLHTSPLCTTNTKEGSNICLTRTDRGWYCDNAGSVSFFPQAETCKVQSNRVFCDTMNSLTLPSEVNLCNVDIFNPKYDCKIMTSKTDVSSSVITSLGAIVSCYGKTKCTASNKNRGIIKTFSNGCDYVSNKGVDTVSVGNTLYYVNKQEGKSLYVKGEPIINFYDPLVFPSDEFDASISQVNEKINQSLAFIRKSDELL

SEQ ID NO: 139 - protein, 466 aa, synthetic construct
QNITEEFYQSTCSAVSKGYLSALRTGWYTSVITIELSNIKENKCNGTDAKVKLIKQFLDKYKNAVTELQLLMQSTPATNNQARGSGSGRSLGFLLGVGSAIASGVAVSKVLHLEGEVNKIKSALLSTNKAVVSLSNGVSVLTSKVLDLKNYIDKQLLPIVNKQSCSISNIETVIEFQQKNNRFLEITREFSVNAGVTTPVSTYMLTNSELLSLINDMPITNDQKKLMSNNVQIVRQQSYSIMSIIKEEVLAYVVQLPLYGVIDTPCWKLHTSPLCTTNTKEGSNICLTRTDRGWYCDNAGSVSFFPQAETCKVQSNRVFCDTMNSLTLPSEVNLCNVDIFNPKYDCKIMTSKTDVSSSVITSLGAIVSCYGKTKCTASNKNRGIIKTFSNGCDYVSNKGVDTVSVGNTLYYVNKQEGKSLYVKGEPIINFYDPLVFPSDEFDASISQVNEKINQSLAFIRKSDELL

SEQ ID NO: 140 - protein, 466 aa, synthetic construct
QNITEEFYQSTCSAVSKGYLSALRTGWYTSVITIELSNIKENKCNGTDAKVKLIKQELDKYKNAVTEFQLLMQSTPATNNQARGSGSGRSLGFLLGVGSAIASGVAVSKVLHLEGEVNKIKSALLSTNKAVVSLSNGVSVLTSKVLDLKNYIDKQLLPIVNKQSCSISNIETVIEFQQKNNRFLEITREFSVNAGVTTPVSTYMLTNSELLSLINDMPITNDQKKLMSNNVQIVRQQSYSIMSIIKEEVLAYVVQLPLYGVIDTPCWKLHTSPLCTTNTKEGSNICLTRTDRGWYCDNAGSVSFFPQAETCKVQSNRVFCDTMNSLTLPSEVNLCNVDIFNPKYDCKIMTSKTDVSSSVITSLGAIVSCYGKTKCTASNKNRGIIKTFSNGCDYVSNKGVDTVSVGNTLYYVNKQEGKSLYVKGEPIINFYDPLVFPSDEFDASISQVNEKINQSLAFIRKSDELL

SEQ ID NO: 141 - protein, 466 aa, synthetic construct
QNITEEFYQSTCSAVSKGYLSALRTGWYTSVITIELSNIKENKCNGTDAKVKLIKQELDKYKNAVTELQLLMQSTPATNNQARGSGSGRSLGFLLGVGSAIASGVAVSKVLHLEGEVNKIKSALLSTNKAVVSLSNGVSVLTSKVLDLKNYIDKQLLPIVNKQSCSISNIETVIEFQQKNNRFLEITREFMVNAGVTTPVSTYMLTNSELLSLINDMPITNDQKKLMSNNVQIVRQQSYSIMSIIKEEVLAYVVQLPLYGVIDTPCWKLHTSPLCTTNTKEGSNICLTRTDRGWYCDNAGSVSFFPQAETCKVQSNRVFCDTMNSLTLPSEVNLCNVDIFNPKYDCKIMTSKTDVSSSVITSLGAIVSCYGKTKCTASNKNRGIIKTFSNGCDYVSNKGVDTVSVGNTLYYVNKQEGKSLYVKGEPIINFYDPLVFPSDEFDASISQVNEKINQSLAFIRKSDELL

SEQ ID NO: 142 - protein, 466 aa, synthetic construct
QNITEEFYQSTCSAVSKGYLSALRTGWYTSVITIELSNIKENKCNGTDAKVKLIKQELDKYKNAVTELQLLMQSTPATNNQARGSGSGRSLGFLLGVGSAIASGVAVSKVLHLEGEVNKIKSALLSTNKAVVSLSNGVSVLTSKVLDLKNYIDKQLLPIVNKQSCSISNIETVIEFQQKMNRLLEIFREFSVNAGVTTPVSTYMLTNSELLSLINDMPITNDQKKLMSNNVQIVRQQSYSIMSIIKEEVLAYVVQLPLYGVIDTPCWKLHTSPLCTTNTKEGSNICLTRTDRGWYCDNAGSVSFFPQAETCKVQSNRVFCDTMNSLTLPSEVNLCNVDIFNPKYDCKIMTSKTDVSSSVITSLGAIVSCYGKTKCTASNKNRGIIKTFSNGCDYVSNKGVDTVSVGNTLYYVNKQEGKSLYVKGEPIINFYDPLVFPSDEFDASISQVNEKINQSLAFIRKSDELL

SEQ ID NO: 143 - protein, 466 aa, synthetic construct
QNITEEFYQSTCSAVSKGYLSALRTGWYTSVITIELSNIKENKCNGTDAKVKLIKQFLDKYKNAVTELQLLMQSTPATNNQARGSGSGRSLGFLLGVGSAIASGVAVSKVLHLEGEVNKIKSALLSTNKAVVSLSNGVSVLTSKVLDLKNYIDKQLLPIVNKQSCSISNIETVIEFQQKNNRLLEIFREFSVNAGVTTPVSTYMLTNSELLSLINDMPITNDQKKLMSNNVQIVRQQSYSIMSIIKEEVLAYVVQLPLYGVIDTPCWKLHTSPLCTTNTKEGSNICLTRTDRGWYCDNAGSVSFFPQAETCKVQSNRVFCDTMNSLTLPSEVNLCNVDIFNPKYDCKIMTSKTDVSSSVITSLGAIVSCYGKTKCTASNKNRGIIKTFSNGCDYVSNKGVDTVSVGNTLYYVNKQEGKSLYVKGEPIINFYDPLVFPSDEFDASISQVNEKINQSLAFIRKSDELL

SEQ ID NO: 144 - protein, 466 aa, synthetic construct
QNITEEFYQSTCSAVSKGYLSALRTGWYTSVITIELSNIKENKCNGTDAKVKLIKQELDKYKNAVTELQLLMQSTPATNNQARGSGSGRSLGFLLGVGSAIASGVAVSKVLHLEGEVNKIKSALLSTNKAVVSLSNGVSVLTSKVMDMKNYIDKQLLPIVNKQSCSISNIETVIEFQQKNNRLLEITREFSVNAGVTTPVSTYMLTNSELLSLINDMPITNDQKKLMSNNVQIVRQQSYSIMSIIKEEVLAYVVQLPLYGVIDTPCWKLHTSPLCTTNTKEGSNICLTRTDRGWYCDNAGSVSFFPQAETCKVQSNRVFCDTMNSLTLPSEVNLCNVDIFNPKYDCKIMTSKTDVSSSVITSLGAIVSCYGKTKCTASNKNRGIIKTFSNGCDYVSNKGVDTVSVGNTLYYVNKQEGKSLYVKGEPIINFYDPLVFPSDEFDASISQVNEKINQSLAFIRKSDELL

SEQ ID NO: 145 - protein, 466 aa, synthetic construct
QNITEEFYQSTCSAVSKGYLSALRTGWYTSVITIELSNIKENKCNGTDAKVKLIKQELDKYKNAVTELQLLMQSTPATNNQARGSGSGRSLGFLLGVGSAIASGVAVSKVLHLEGEVNKIKSALLSTNKAVVSLSNGVSVLTVKVMDMKNYIDKQLLPIVNKQSCSISNIETVIEFQQKNNRLLEITREFSVNAGVTTPVSTYMLTNSELLSLINDMPITNDQKKLMSNNVQIVRQQSYSIMSIIKEEVLAYVVQLPLYGVIDTPCWKLHTSPLCTTNTKEGSNICLTRTDRGWYCDNAGSVSFFPQAETCKVQSNRVFCDTMNSLTLPSEVNLCNVDIFNPKYDCKIMTSKTDVSSSVITSLGAIVSCYGKTKCTASNKNRGIIKTFSNGCDYVSNKGVDTVSVGNTLYYVNKQEGKSLYVKGEPIINFYDPLVFPSDEFDASISQVNEKINQSLAFIRKSDELL

SEQ ID NO: 146 - protein, 466 aa, synthetic construct
QNITEEFYQSTCSAVSKGYLSALRTGWYTSVITIELSNIKENKCNGTDAKVKLIKQELDKYKNAVTELQLLMQSTPATNNQARGSGSGRSLGFLLGVGSAIASGVAVSKVLHLEGEVNKIKSALLSTNKAVVSLSNGVSVLTSKVMDLKNYMDKQLLPIVNKQSCSISNIETVIEFQQKNNRLLEITREFSVNAGVTTPVSTYMLTNSELLSLINDMPITNDQKKLMSNNVQIVRQQSYSIMSIIKEEVLAYVVQLPLYGVIDTPCWKLHTSPLCTTNTKEGSNICLTRTDRGWYCDNAGSVSFFPQAETCKVQSNRVFCDTMNSLTLPSEVNLCNVDIFNPKYDCKIMTSKTDVSSSVITSLGAIVSCYGKTKCTASNKNRGIIKTFSNGCDYVSNKGVDTVSVGNTLYYVNKQEGKSLYVKGEPIINFYDPLVFPSDEFDASISQVNEKINQSLAFIRKSDELL

SEQ ID NO: 147 - protein, 466 aa, synthetic construct
QNITEEFYQSTCSAVSKGYLSALRTGWYTSVITIELSNIKENKCNGTDAKVKLIKQELDKYKNAVTELQLLMQSTPATNNQARGSGSGRSLGFLLGVGSAIASGVAVSKVLHLEGEVNKIKSALLSTNKAVVSLSNGVSVLTSKVMDLKNYFDKQLLPIVNKQSCSISNIETVIEFQQKNNRLLEITREFSVNAGVTTPVSTYMLTNSELLSLINDMPITNDQKKLMSNNVQIVRQQSYSIMSIIKEEVLAYVVQLPLYGVIDTPCWKLHTSPLCTTNTKEGSNICLTRTDRGWYCDNAGSVSFFPQAETCKVQSNRVFCDTMNSLTLPSEVNLCNVDIFNPKYDCKIMTSKTDVSSSVITSLGAIVSCYGKTKCTASNKNRGIIKTFSNGCDYVSNKGVDTVSVGNTLYYVNKQEGKSLYVKGEPIINFYDPLVFPSDEFDASISQVNEKINQSLAFIRKSDELL

SEQ ID NO: 148 - protein, 466 aa, synthetic construct
QNITEEFYQSTCSAVSKGYLSALRTGWYTSVITIELSNIKENKCNGTDAKVKLIKQELDKYKNAVTELQLLMQSTPATNNQARGSGSGRSLGFMLGVGSAIASGVAVSKVLHLEGEVNKIKSALLSTNKAVVSLSNGVSVLTSKVLDLKNYIDKQLLPIVNKQSCSISNIETVIEFQQKNNRLLEITREFSVNAGVTTPVSTYMLTNSELLSLINDMPITNDQKKLMSNNVQIVRQQSYSIMSIIKEEVLAYVVQLPLYGVIDTPCWKLHTSPLCTTNTKEGSNICLTRTDRGWYCDNAGSVSFFPQAETCKVQSNRVFCDTMNSMTLPSEVNLCNVDIFNPKYDCKIMTSKTDVSSSVITSLGAIVSCYGKTKCTASNKNRGIIKTFSNGCDYVSNKGVDTVSVGNTLYYVNKQEGKSLYVKGEPIINFYDPLVFPSDEFDASISQVNEKINQSLAFIRKSDELL

SEQ ID NO: 149 - protein, 466 aa, synthetic construct
QNITEEFYQSTCSAVSKGYLSALRTGWYTSVITIELSNIKENKCNGTDAKVKLIKQELDKYKNAVTELQLLMQSTPATNNQARGSGSGRSLGFFLGVGSAIASGVAVSKVLHLEGEVNKIKSALLSTNKAVVSLSNGVSVLTSKVLDLKNYIDKQLLPIVNKQSCSISNIETVIEFQQKNNRLLEITREFSVNAGVTTPVSTYMLTNSELLSLINDMPITNDQKKLMSNNVQIVRQQSYSIMSIIKEEVLAYVVQLPLYGVIDTPCWKLHTSPLCTTNTKEGSNICLTRTDRGWYCDNAGSVSFFPQAETCKVQSNRVFCDTMNSFTLPSEVNLCNVDIFNPKYDCKIMTSKTDVSSSVITSLGAIVSCYGKTKCTASNKNRGIIKTFSNGCDYVSNKGVDTVSVGNTLYYVNKQEGKSLYVKGEPIINFYDPLVFPSDEFDASISQVNEKINQSLAFIRKSDELL

SEQ ID NO: 150 - protein, 466 aa, synthetic construct
QNITEEFYQSTCSAVSKGYLSALRTGWYTSVITIELSNIKENKCNGTDAKVKLIKQCLDKYKNAVTELQLLMQSTPATNNQARGSGSGRSLGFLLGVGSAIASGVAVSKVLHLEGEVNKIKSALLSTNKAVVSLSNGVSVLTSKVLDLKNYIDKQLLPIVNKQSCSISNIETVIEFCQKNNRLLEITREFSVNAGVTTPVSTYMLTNSELLSLINDMPITNDQKKLMSNNVQIVRQQSYSIMSIIKEEVLAYVVQLPLYGVIDTPCWKLHTSPLCTTNTKEGSNICLTRTDRGWYCDNAGSVSFFPQAETCKVQSNRVFCDTMNSLTLPSEVNLCNVDIFNPKYDCKIMTSKTDVSSSVITSLGAIVSCYGKTKCTASNKNRGIIKTFSNGCDYVSNKGVDTVSVGNTLYYVNKQEGKSLYVKGEPIINFYDPLVFPSDEFDASISQVNEKINQSLAFIRKSDELL

SEQ ID NO: 151 - protein, 466 aa, synthetic construct
QNITEEFYQSTCSAVSKGYLSALRTGWYTSVITIELSNIKENKCNGTDAKVKLIKQELDKYKNAVTCLQLLMQSTPATNNQARGSGSGRSLGFLLGVGSAIASGVAVSKVLHLEGEVNKIKSALLSTNKAVVSLSNGVSVLTSKVLDLKNYIDKQLLPIVNKQSCSISNIETVIEFQQKNNRLLEITREFCVNAGVTTPVSTYMLTNSELLSLINDMPITNDQKKLMSNNVQIVRQQSYSIMSIIKEEVLAYVVQLPLYGVIDTPCWKLHTSPLCTTNTKEGSNICLTRTDRGWYCDNAGSVSFFPQAETCKVQSNRVFCDTMNSLTLPSEVNLCNVDIFNPKYDCKIMTSKTDVSSSVITSLGAIVSCYGKTKCTASNKNRGIIKTFSNGCDYVSNKGVDTVSVGNTLYYVNKQEGKSLYVKGEPIINFYDPLVFPSDEFDASISQVNEKINQSLAFIRKSDELL

SEQ ID NO: 152 - protein, 466 aa, synthetic construct
QNITEEFYQSTCSAVSKGYLSALRTGWYTSVITIELSNIKENKCNGTDAKVKLCKQELDKYKNAVTELQLLMQSTPATNNQARGSGSGRSLGFLLGVGSAIASGVAVSKVLHLEGEVNKIKSALLSTNKAVVSLSNGVSVLTSKVLDLKNYIDKQLLPIVNKQSCSISNIETCIEFQQKNNRLLEITREFSVNAGVTTPVSTYMLTNSELLSLINDMPITNDQKKLMSNNVQIVRQQSYSIMSIIKEEVLAYVVQLPLYGVIDTPCWKLHTSPLCTTNTKEGSNICLTRTDRGWYCDNAGSVSFFPQAETCKVQSNRVFCDTMNSLTLPSEVNLCNVDIFNPKYDCKIMTSKTDVSSSVITSLGAIVSCYGKTKCTASNKNRGIIKTFSNGCDYVSNKGVDTVSVGNTLYYVNKQEGKSLYVKGEPIINFYDPLVFPSDEFDASISQVNEKINQSLAFIRKSDELL

SEQ ID NO: 153 - protein, 466 aa, synthetic construct
QNITEEFYQSTCSAVSKGYLSALRTGWYTSVITIELSNIKENKCNGTDAKVKLIKQELDKYKNAVTELQLLCQSTPATNNQARGSGSGRSLGFLLGVGSAIASGVAVSKVLHLEGEVNKIKSALLSTNKAVVSLSNGVSVLTSKVLDLKNYIDKQLLPIVNKQSCSISNIETVIEFQQKNNRLLEITREFSVNAGVTTPVSTYMLTNSELLSLINDMPITNDQKKLMSNNVQIVRQQSYSIMSCIKEEVLAYVVQLPLYGVIDTPCWKLHTSPLCTTNTKEGSNICLTRTDRGWYCDNAGSVSFFPQAETCKVQSNRVFCDTMNSLTLPSEVNLCNVDIFNPKYDCKIMTSKTDVSSSVITSLGAIVSCYGKTKCTASNKNRGIIKTFSNGCDYVSNKGVDTVSVGNTLYYVNKQEGKSLYVKGEPIINFYDPLVFPSDEFDASISQVNEKINQSLAFIRKSDELL

SEQ ID NO: 154 - protein, 466 aa, synthetic construct
QNITEEFYQSTCSAVSKGYLSALRTGWYTSVITIELSNIKENKCNGTDAKVKLIKQELDKYKNAVTECQLLMQSTPATNNQARGSGSGRSLGFLLGVGSAIASGVAVSKVLHLEGEVNKIKSALLSTNKAVVSLSNGVSVLTSKVLDLKNYIDKQLLPIVNKQSCSISNIETVIEFQQKNNRLLEICREFSVNAGVTTPVSTYMLTNSELLSLINDMPITNDQKKLMSNNVQIVRQQSYSIMSIIKEEVLAYVVQLPLYGVIDTPCWKLHTSPLCTTNTKEGSNICLTRTDRGWYCDNAGSVSFFPQAETCKVQSNRVFCDTMNSLTLPSEVNLCNVDIFNPKYDCKIMTSKTDVSSSVITSLGAIVSCYGKTKCTASNKNRGIIKTFSNGCDYVSNKGVDTVSVGNTLYYVNKQEGKSLYVKGEPIINFYDPLVFPSDEFDASISQVNEKINQSLAFIRKSDELL

SEQ ID NO: 155 - protein, 466 aa, synthetic construct
QNITEEFYQSTCSAVSKGYLSALRTGWYTSVITIELSNIKENKCNGTDAKVKLIKQELDKYKNAVTCLQLLMQSTPATNNQARGSGSGRSLGFLLGVGSAIASGVAVSKVLHLEGEVNKIKSALLSTNKAVVSLSNGVSVLTSKVLDLKNYIDKQLLPIVNKQSCSISNIETVIEFQQKNNRLLEICREFSVNAGVTTPVSTYMLTNSELLSLINDMPITNDQKKLMSNNVQIVRQQSYSIMSIIKEEVLAYVVQLPLYGVIDTPCWKLHTSPLCTTNTKEGSNICLTRTDRGWYCDNAGSVSFFPQAETCKVQSNRVFCDTMNSLTLPSEVNLCNVDIFNPKYDCKIMTSKTDVSSSVITSLGAIVSCYGKTKCTASNKNRGIIKTFSNGCDYVSNKGVDTVSVGNTLYYVNKQEGKSLYVKGEPIINFYDPLVFPSDEFDASISQVNEKINQSLAFIRKSDELL

SEQ ID NO: 156 - protein, 466 aa, synthetic construct
QNITEEFYQSTCSAVSKGYLSALRTGWYTSVITIELSNIKENKCNGTDAKVKLIKQELDKYKNAVTELQLLMQSTPATNNQARGSGSGRSLGFLLGVGSAIASGVAVSKVLHLEGEVNKIKSALLSTNKAVVSLSNGVSVLTSKVLDLKNYIDKQLLPIVNKQSCSISNIETVIEFQQKMNRFLEITREFSVNAGVTTPVSTYMLTNSELLSLINDMPITNDQKKLMSNNVQIVRQQSYSIMSIIKEEVLAYVVQLPLYGVIDTPCWKLHTSPLCTTNTKEGSNICLTRTDRGWYCDNAGSVSFFPQAETCKVQSNRVFCDTMNSLTLPSEVNLCNVDIFNPKYDCKIMTSKTDVSSSVITSLGAIVSCYGKTKCTASNKNRGIIKTFSNGCDYVSNKGVDTVSVGNTLYYVNKQEGKSLYVKGEPIINFYDPLVFPSDEFDASISQVNEKINQSLAFIRKSDELL

SEQ ID NO: 157 - protein, 466 aa, synthetic construct
QNITEEFYQSTCSAVSKGYLSALRTGWYTSVITIELSNIKENKCNGTDAKVKLIKQELDKYKNAVTELQLLMQSTPATNNQARGSGSGRSLGFLLGVGSAIASGVAVSKVLHLEGEVNKIKSALLSTNKAVVSLSNGVSVLTVKVMDLKNYIDKQLLPIVNKQSCSISNIETVIEFQQKMNRFLEITREFSVNAGVTTPVSTYMLTNSELLSLINDMPITNDQKKLMSNNVQIVRQQSYSIMSIIKEEVLAYVVQLPLYGVIDTPCWKLHTSPLCTTNTKEGSNICLTRTDRGWYCDNAGSVSFFPQAETCKVQSNRVFCDTMNSLTLPSEVNLCNVDIFNPKYDCKIMTSKTDVSSSVITSLGAIVSCYGKTKCTASNKNRGIIKTFSNGCDYVSNKGVDTVSVGNTLYYVNKQEGKSLYVKGEPIINFYDPLVFPSDEFDASISQVNEKINQSLAFIRKSDELL

SEQ ID NO: 158 - protein, 466 aa, synthetic construct
QNITEEFYQSTCSAVSKGYLSALRTGWYTSVITIELSNIKENKCNGTDAKVKLIKQELDKYKNAVTELQLLMQSTPATNNQARGSGSGRSLGFLLGVGSAIASGVAVSKVLHLEGEVNKIKSALLSTNKAVVSLSNGVSVLTSKVLDLKNYIDKQLLPIVNKQSCSISNIETVIEFQQKMNRFLEITREFSVNAGVTTPVSTYMLTNSELLSLINDMPITNDQKKLMSNNVQIVRQQSYSIMSIIKEEVLAYVVQLPLYGVIDTPCWKLHTSPLCTTNTKEGSNICLTRTDRGWYCDNAGSVSFFPQAETCKVQSNRVFCDTMNSLTLPSEVNLCNVDIFNPKYDCKIMTSKTDVSSSVITSLGAIVSCYGKTKCTASNKNRGIIKTFSNGCDYVSNKGVDTVSVGNTLYYVNKQEGKSLYVKGEPIINFYDPLVFPSDEFDASISQVNEKINQSLAFIRKMDELL

SEQ ID NO: 159 - protein, 466 aa, synthetic construct
QNITEEFYQSTCSAVSKGYLSALRTGWYTSVITIELSNIKENKCNGTDAKVKLIKQELDKYKNAVTELQLLMQSTPATNNQARGSGSGRSLGFLLGVGSAIASGVAVSKVLHLEGEVNKIKSALLSTNKAVVSLSNGVSVLTSKVLDLKNYIDKQLLPIVNKQSCSISNIETVIEFQQKMNRFLEITREFSVNAGVTTPVSTYMLTNSELLSLINDMPITNDQKKLMSNNVQIVRQQSYSIMSIIKEEVLAYVVQLPLYGVIDTPCWKLHTSPLCTTNTKEGSNICLTRTDRGWYCDNAGSVSFFPQAETCKVQSNRVFCDTMNSLTLPSEVNLCNVDIFNPKYDCKIMTSKTDVSSSVITSLGAIVSCYGKTKCTASNKNRGIIKTFSNGCDYVSNKGVDTVSVGNTLYYVNKQEGKSLYVKGEPIINFYDPLVFPSDEFDASISQVNEKINQSLAFIRKFDELL

SEQ ID NO: 160 - protein, 466 aa, synthetic construct
QNITEEFYQSTCSAVSKGYLSALRTGWYTSVITIELSNIKENKCNGTDAKVKLIKQELDKYKNAVTELQLLMQSTPATNNQARGSGSGRSLGFLLGVGSAIASGVAVSKVLHLEGEVNKIKSALLSTNKAVVSLSNGVSVLTSKVLDLKNYIDKQLLPIVNKQSCSISNIETVIEFQQKMNRFLEITREFSVNAGVTTPVSTYMLTNSELLSLINDMPITNDQKKLMSNNVQIVRQQSYSIMSIIKEEVLAYVVQLPLYGVIDTPCWKLHTSPLCTTNTKEGSNICLTRTDRGWYCDNAGSVSFFPQAETCKVQSNRVFCDTMNSLTLPSEVNLCNVDIFNPKYDCKIMTSKTDVSSSVITSLGAIVSCYGKTKCTASNKNRGIIKTFSNGCDYVSNKGVDTVSVGNTLYYVNKQEGKSLYVKGEPIINFYDPLVFPSDEFDASISQVNEKINQSLAFIRKLDELL

SEQ ID NO: 161 - protein, 466 aa, synthetic construct
QNITEEFYQSTCSAVSKGYLSALRTGWYTSVITIELSNIKENKCNGTDAKVKLIKQELDKYKNAVTELQLLMQSTPATNNQARGSGSGRSLGFLLGVGSAIASGVAVSKVLHLEGEVNKIKSALLSTNKAVVSLSNGVSVLTSKVLDLKNYIDKQLLPIVNKQSCSISNIETVIEFQQKMNRFLEITREFSVNAGVTTPVSTYMLTNSELLSLINDMPITNDQKKLMSNNVQIVRQQSYSIMSIIKEEVLAYVVQLPLYGVIDTPCWKLHTSPLCTTNTKEGSNICLTRTDRGWYCDNAGSVSFFPQAETCKVQSNRVFCDTMNSLTLPSEVNLCNVDIFNPKYDCKIMTSKTDVSSSVITSLGAIVSCYGKTKCTASNKNRGIIKTFSNGCDYVSNKGVDTVSVGNTLYYVNKQEGKSLYVKGEPIINFYDPLVFPSDEFDASISQVNEKINQSLAWIRKSDELL

SEQ ID NO: 162 - protein, 465 aa, synthetic construct
QNITEEFYQSTCSAVSKGYLSALRTGWYTSVITIELSNIKENKCNGTDAKVKLIKQELDKYKNAVTELQLLMQSTPATNNQARGSGSGRSLGFLLGVGSAIASGVAVSKVLHLEGEVNKIKSALLSTNKAVVSLSNGVSVLTSKVLDLKNYIDKQLLPIVNKQSCSISNIETVIEFQQKMNRFLEITREFSVNAGVTTPVSTYMLTNSELLSLINDMPITNDQKKLMSNNVQIVRQQSYSIMSIIKEEVLAYVVQLPLYGVIDTPCWKLHTSPLCTTNTKEGSNICLTRTDRGWYCDNAGSVSFFPQAETCKVQSNRVFCDTMNSLTLSEVNLCNVDIFNPKYDCKIMTSKTDVSSSVITSLGAIVSCYGKTKCTASNKNRGIIKTFSNGCDYVSNKGVDTVSVGNTLYYVNKQEGKSLYVKGEPIINFYDPLVFPSDEFDASISQVNEKINQYLAFIRKSDELL

SEQ ID NO: 163 - protein, 466 aa, synthetic construct
QNITEEFYQSTCSAVSKGYLSALRTGWYTSVITIELSNIKENKCNGTDAKVKLIKQELDKYKNAVTELQLLMQSTPATNNQARGSGSGRSLGFLLGVGSAIASGVAVSKVLHLEGEVNKIKSALLSTNKAVVSLSNGVSVLTSKVLDLKNYIDKQLLPIVNKQSCSISNIETVIEFQQKMNRFLEITREFSVNAGVTTPVSTYMLTNSELLSLINDMPITNDQKKLMSNNVQIVRQQSYSIMSIIKEEVLAYVVQLPLYGVIDTPCWKLHTSPLCTTNTKEGSNICLTRTDRGWYCDNAGSVSFFPQAETCKVQSNRVFCDTMNSLTLPSEVNLCNVDIFNPKYDCKIMTSKTDVSSSVITSLGAIVSCYGKTKCTASNKNRGIIKTFSNGCDYVSNKGVDTVSVGNTLYYVNKQEGKSLYVKGEPIINFYDPLVFPSDEFDASISQVNEKINQSLAWIRKLDELL

SEQ ID NO: 164 - protein, 466 aa, synthetic construct
QNITEEFYQSTCSAVSKGYLSALRTGWYTSVITIELSNIKENKCNGTDAKVKLIKQELDKYKNAVTELQLLMQSTPATNNQARGSGSGRSLGFLLGVGSAIASGVAVSKVLHLEGEVNKIKSALLSTNKAVVSLSNGVSVLTSKVLDLKNYIDKQLLPIVNKQSCSISNIETVIEFQQKMNRFLEITREFSVNAGVTTPVSTYMLTNSELLSLINDMPITNDQKKLMSNNVQIVRQQSYSIMSIIKEEVLAYVVQLPLYGVIDTPCWKLHTSPLCTTNTKEGSNICLTRTDRGWYCDNAGSVSFFPQAETCKVQSNRVFCDTMNSLTLPSEVNLCNVDIFNPKYDCKIMTSKTDVSSSVITSLGAIVSCYGKTKCTASNKNRGIIKTFSNGCDYVSNKGVDTVSVGNTLYYVNKQEGKSLYVKGEPIINFYDPLVFPSDEFDASISQVNEKINMSLAFIRKFDELL

SEQ ID NO: 165 - protein, 466 aa, synthetic construct
QNITEEFYQSTCSAVSKGYLSALRTGWYTSVITIELSNIKENKCNGTDAKVKLIKQELDKYKNAVTELQLLMQSTPATNNQARGSGSGRSLGFLLGVGSAIASGVAVSKVLHLEGEVNKIKSALLSTNKAVVSLSNGVSVLTVKVMDLKNYIDKQLLPIVNKQSCSISNIETVIEFQQKMNRFLEITREFSVNAGVTTPVSTYMLTNSELLSLINDMPITNDQKKLMSNNVQIVRQQSYSIMSIIKEEVLAYVVQLPLYGVIDTPCWKLHTSPLCTTNTKEGSNICLTRTDRGWYCDNAGSVSFFPQAETCKVQSNRVFCDTMNSLTLPSEVNLCNVDIFNPKYDCKIMTSKTDVSSSVITSLGAIVSCYGKTKCTASNKNRGIIKTFSNGCDYVSNKGVDTVSVGNTLYYVNKQEGKSLYVKGEPIINFYDPLVFPSDEFDASISQVNEKINQSLAWIRKLDELL

SEQ ID NO: 166 - protein, 466 aa, synthetic construct
QNITEEFYQSTCSAVSKGYLSALRTGWYTSVITIELSNIKENKCNGTDAKVKLIKQELDKYKNAVTELQLLMQSTPATNNQARGSGSGRSLGFLLGVGSAIASGVAVSKVLHLEGEVNKIKSALLSTNKAVVSLSNGVSVLTVKVMDLKNYIDKQLLPIVNKQSCSISNIETVIEFQQKMNRFLEITREFSVNAGVTTPVSTYMLTNSELLSLINDMPITNDQKKLMSNNVQIVRQQSYSIMSIIKEEVLAYVVQLPLYGVIDTPCWKLHTSPLCTTNTKEGSNICLTRTDRGWYCDNAGSVSFFPQAETCKVQSNRVFCDTMNSLTLPSEVNLCNVDIFNPKYDCKIMTSKTDVSSSVITSLGAIVSCYGKTKCTASNKNRGIIKTFSNGCDYVSNKGVDTVSVGNTLYYVNKQEGKSLYVKGEPIINFYDPLVFPSDEFDASISQVNEKINMSLAFIRKFDELL